European Patent Application EP 4 365 193 A1, published May 8, 2024. Title: CHIMERIC POLYPEPTIDE FOR REGULATING CELL PHYSIOLOGICAL ACTIVITY. Applicant: CARSGEN THERAPEUTICS CO., LTD. The sequence listing filed with the application follows.

SEQUENCE LISTING (110 sequences)

SEQ ID NO: 1 - protein, 218 aa, Amino acid of Jagged2 extracellular region
EVIGFGRSCWSRGTPFPHGSSWVEDCNSCRCLDGRRDCSKVWCGWKPCLLAGQPEALSAQCPLGQRCLEKAPGQCLRPPCEAWGECGAEEPPSTPCLPRSGHLDNNCARLTLHFNRDHVPQGTTVGAICSGIRSLPATRAVARDRLLVLLCDRASSGASAVEVAVSFSPARDLPDSSLIQGAAHAIVAAITQRGNSSLLLAVTEVKVETVVTGGSSTG

SEQ ID NO: 2 - DNA, 654 bp, Amino acid of Jagged2 extracellular region
gaagtgatcgggttcgggagatcctgctggtcccggggcactccgttcccacacggaagctcctgggtggaagactgcaacagctgccgctgcctggatggccgccgtgactgcagcaaggtgtggtgcggatggaagccttgtctgctggccggccagcccgaggccctgagcgcccagtgcccactggggcaaaggtgcctggagaaggccccaggccagtgtctgcgaccaccctgtgaggcctggggggagtgcggcgcagaagagccaccgagcaccccctgcctgccacgctccggccacctggacaataactgtgcccgcctcaccttgcatttcaaccgtgaccacgtgccccagggcaccacggtgggcgccatttgctccgggatccgctccctgccagccacaagggctgtggcacgggaccgcctgctggtgttgctttgcgaccgggcgtcctcgggggccagtgctgtggaggtggccgtgtccttcagccctgccagggacctgcctgacagcagcctgatccagggcgcggcccacgccatcgtggccgccatcacccagcgggggaacagctcactgctcctggctgtcaccgaggtcaaggtggagacggttgttacgggcggctcttccacaggt

SEQ ID NO: 3 - protein, 65 aa, Amino acid of EphrinB2 extracellular region(full length)
GQDASSAGSTRNKDPTRRPELEAGTNGRSSTTSPFVKPNPGSSTDGNSAGHSGNNILGSEVALFA

SEQ ID NO: 4 - DNA, 195 bp, Nucleotide of EphrinB2 extracellular region (full length)
ggacaagatgcaagttctgctggatcaaccaggaataaagatccaacaagacgtccagaactagaagctggtacaaatggaagaagttcgacaacaagtccctttgtaaaaccaaatccaggttctagcacagacggcaacagcgccggacattcggggaacaacatcctcggttccgaagtggccttatttgca

SEQ ID NO: 5 - protein, 54 aa, Amino acid of EphrinB2-del1 extracellular region
GQDATRRPELEAGTNGRSSTTSPFVKPNPGSSTDGNSAGHSGNNILGSEVALFA

SEQ ID NO: 6 - DNA, 162 bp, Nucleotide of EphrinB2-del1 extracellular region
ggacaagatgcaacaagacgtccagaactagaagctggtacaaatggaagaagttcgacaacaagtccctttgtaaaaccaaatccaggttctagcacagacggcaacagcgccggacattcggggaacaacatcctcggttccgaagtggccttatttgca

SEQ ID NO: 7 - protein, 52 aa, Amino acid of EphrinB2-del2 extracellular region
GQDASSAGSTRNKDPTRRPSPFVKPNPGSSTDGNSAGHSGNNILGSEVALFA

SEQ ID NO: 8 - DNA, 156 bp, Nucleic acid of EphrinB2-del2 extracellular region
ggacaagatgcaagttctgctggatcaaccaggaataaagatccaacaagacgtccaagtccctttgtaaaaccaaatccaggttctagcacagacggcaacagcgccggacattcggggaacaacatcctcggttccgaagtggccttatttgca

SEQ ID NO: 9 - protein, 41 aa, Amino acid of EphrinB2-del3 extracellular region
GQDASSAGSTRNKDPTRRPELEAGTNGRSSTTSPSEVALFA

SEQ ID NO: 10 - DNA, 123 bp, Nucleotide of EphrinB2-del3 extracellular region
ggacaagatgcaagttctgctggatcaaccaggaataaagatccaacaagacgtccagaactagaagctggtacaaatggaagaagttcgacaacaagtccctccgaagtggccttatttgca

SEQ ID NO: 11 - protein, 26 aa, Amino acid of EphrinB2-del23 extracellular region
GQDASSAGSTRNKDPTRRPSEVALFA

SEQ ID NO: 12 - DNA, 78 bp, Nucleotide of EphrinB2-del23 extracellular region
ggacaagatgcaagttctgctggatcaaccaggaataaagatccaacaagacgtccatccgaagtggccttatttgca

SEQ ID NO: 13 - protein, 27 aa, Mouse Notch1 transmembrane region
LMYVAAAAFVLLFFVGCGVLLSRKRRR

SEQ ID NO: 14 - protein, 29 aa, Mouse Notch2 transmembrane region
LLYLLAVAVVIILFFILLGVIMAKRKRKH

SEQ ID NO: 15 - protein, 29 aa, Mouse Notch3 transmembrane region
LLPLLVAGAVFLLIIFILGVMVARRKREH

SEQ ID NO: 16 - protein, 31 aa, Mouse Notch4 transmembrane region
PILCSPVVGVLLLALGALLVLQLIRRRRREH

SEQ ID NO: 17 - protein, 27 aa, Human Notch1 transmembrane region
FMYVAAAAFVLLFFVGCGVLLSRKRRR

SEQ ID NO: 18 - protein, 29 aa, Human Notch2 transmembrane region
LLYLLAVAVVIILFIILLGVIMAKRKRKH

SEQ ID NO: 19 - protein, 28 aa, Human Notch3 transmembrane region
LPLLVAGAVLLLVILVLGVMVARRKREH

SEQ ID NO: 20 - protein, 31 aa, Human Notch4 transmembrane region
PVLCSPVAGVILLALGALLVLQLIRRRRREH

SEQ ID NO: 21 - protein, 28 aa, APLP2 transmembrane region
SALIGLLVIAVAIATVIVISLVMLRKRQ

SEQ ID NO: 22 - protein, 5 aa, Notch1STS
RKRRR

SEQ ID NO: 23 - protein, 6 aa, Notch2STS
KRKRKH

SEQ ID NO: 24 - protein, 6 aa, Notch3STS
RRKREH

SEQ ID NO: 25 - protein, 7 aa, Notch4STS
RRRRREH

SEQ ID NO: 26 - protein, 4 aa, STS of APLP2
RKRQ

SEQ ID NO: 27 - protein, 211 aa, GAL4-VP64
MKLLSSIEQACDICRLKKLKCSKEKPKCAKCLKNNWECRYSPKTKRSPLTRAHLTEVESRLERLEQLFLLIFPREDLDMILKMDSLQDIKALLTGLFVQDNVNKDAVTDRLASVETDMPLTLRQHRISATSSSEESSNKGQRQLTVSAAAGGSGGSGGSDALDDFDLDMLGSDALDDFDLDMLGSDALDDFDLDMLGSDALDDFDLDMLGS

SEQ ID NO: 28 - protein, 245 aa, Receptor regulatory domain of synJagged2EC
EVIGFGRSCWSRGTPFPHGSSWVEDCNSCRCLDGRRDCSKVWCGWKPCLLAGQPEALSAQCPLGQRCLEKAPGQCLRPPCEAWGECGAEEPPSTPCLPRSGHLDNNCARLTLHFNRDHVPQGTTVGAICSGIRSLPATRAVARDRLLVLLCDRASSGASAVEVAVSFSPARDLPDSSLIQGAAHAIVAAITQRGNSSLLLAVTEVKVETVVTGGSSTGLMYVAAAAFVLLFFVGCGVLLSRKRRR

SEQ ID NO: 29 - protein, 92 aa, Receptor regulatory domain of synEphrinB2EC
GQDASSAGSTRNKDPTRRPELEAGTNGRSSTTSPFVKPNPGSSTDGNSAGHSGNNILGSEVALFALMYVAAAAFVLLFFVGCGVLLSRKRRR

SEQ ID NO: 30 - protein, 93 aa, Receptor regulatory domain of synEphrinB2EC-2
GQDASSAGSTRNKDPTRRPELEAGTNGRSSTTSPFVKPNPGSSTDGNSAGHSGNNILGSEVALFALMYVAAAAFVLLFFVGCGVLLSKRKRKH

SEQ ID NO: 31 - protein, 93 aa, Receptor regulatory domain of synEphrinB2EC-3
GQDASSAGSTRNKDPTRRPELEAGTNGRSSTTSPFVKPNPGSSTDGNSAGHSGNNILGSEVALFALMYVAAAAFVLLFFVGCGVLLSRRKREH

SEQ ID NO: 32 - protein, 94 aa, Receptor regulatory domain of synEphrinB2EC-4
GQDASSAGSTRNKDPTRRPELEAGTNGRSSTTSPFVKPNPGSSTDGNSAGHSGNNILGSEVALFALMYVAAAAFVLLFFVGCGVLLSRRRRREH

SEQ ID NO: 33 - protein, 94 aa, Receptor regulatory domain of synEphrinB2EC-5
GQDASSAGSTRNKDPTRRPELEAGTNGRSSTTSPFVKPNPGSSTDGNSAGHSGNNILGSEVALFALLYLLAVAVVIILFIILLGVIMAKRKRKH

SEQ ID NO: 34 - protein, 93 aa, Receptor regulatory domain of synEphrinB2EC-6
GQDASSAGSTRNKDPTRRPELEAGTNGRSSTTSPFVKPNPGSSTDGNSAGHSGNNILGSEVALFALPLLVAGAVLLLVILVLGVMVARRKREH

SEQ ID NO: 35 - protein, 96 aa, Receptor regulatory domain of synEphrinB2EC-7
GQDASSAGSTRNKDPTRRPELEAGTNGRSSTTSPFVKPNPGSSTDGNSAGHSGNNILGSEVALFAPVLCSPVAGVILLALGALLVLQLIRRRRREH

SEQ ID NO: 36 - protein, 93 aa, Receptor regulatory domain of synEphrinB2EC-APLP2TM
GQDASSAGSTRNKDPTRRPELEAGTNGRSSTTSPFVKPNPGSSTDGNSAGHSGNNILGSEVALFASALIGLLVIAVAIATVIVISLVMLRKRQ

SEQ ID NO: 37 - protein, 81 aa, Receptor regulatory domain of synEphrinB2EC-del1
GQDATRRPELEAGTNGRSSTTSPFVKPNPGSSTDGNSAGHSGNNILGSEVALFALMYVAAAAFVLLFFVGCGVLLSRKRRR

SEQ ID NO: 38 - protein, 79 aa, Receptor regulatory domain of synEphrinB2EC-del2
GQDASSAGSTRNKDPTRRPSPFVKPNPGSSTDGNSAGHSGNNILGSEVALFALMYVAAAAFVLLFFVGCGVLLSRKRRR

SEQ ID NO: 39 - protein, 68 aa, Receptor regulatory domain of synEphrinB2EC-del3
GQDASSAGSTRNKDPTRRPELEAGTNGRSSTTSPSEVALFALMYVAAAAFVLLFFVGCGVLLSRKRRR

SEQ ID NO: 40 - protein, 69 aa, Receptor regulatory domain of synEphrinB2EC-del3-2
GQDASSAGSTRNKDPTRRPELEAGTNGRSSTTSPSEVALFALMYVAAAAFVLLFFVGCGVLLSKRKRKH

SEQ ID NO: 41 - protein, 53 aa, Receptor regulatory domain of synEphrinB2EC-del23
GQDASSAGSTRNKDPTRRPSEVALFALMYVAAAAFVLLFFVGCGVLLSRKRRR

SEQ ID NO: 42 - protein, 243 aa, antiGPC3-scFv
EVQLVQSGAEVKKPGASVKVSCKASGYTFSDYEMHWVRQAPGQGLEWMGAIHPGSGDTAYNQRFKGRVTITADKSTSTAYMELSSLRSEDTAVYYCARFYSYAYWGQGTLVTVSAGGGGSGGGGSGGGGSDIVMTQTPLSLPVTPGEPASISCRSSQSLVHSNGNTYLQWYLQKPGQSPQLLIYKVSNRFSGVPDRFSGSGSGTDFTLKISRVEAEDVGVYYCSQSIYVPYTFGQGTKLEIKR

SEQ ID NO: 43 - protein, 239 aa, antiEGFRvIII-scFv
DIQMTQSPSSLSASVGDRVTITCHASQDINVNIGWLQQKPGKAFKGLIYHGKNLEDGVPSRFSGSGSGTDFTLTISSLQPEDFATYYCNQYENIPLTFGQGTKVEIKRGGGGSGGGGSGGGGSDVQLVESGGGLVQPGGSLRLSCAVSGYSITSDYAWNWIRQAPGKGLEWLGYISYRGRTQYNPSLKSRISITRDNSKNTFFLQLNSLRAEDTAVYYCARMGKNWDYWGQGTLVTVSS

SEQ ID NO: 44 - protein, 247 aa, antiMesothelin-scFv
QMQLVQSGAEVKKPGASVKVSCKASGYTFTSYYMHWVRQAPGQGLEWMGIINPSGGSTSYAQKFQGRVTMTRDTSTSTVYMELSSLRSEDTAVYYCASSRSGTTVVNHDAFDIWGKGTTVTVSSGGGGSGGGGSGGGGSDIQLTQSPSSLSASVGDRVTITCRASQVISRALAWYQQTPGKPPKLLIYDASNLQSGVPSRFSGSGSGTDFTLTISRLQPEDFATYYCQQFNSYPLTFGGGTKLEIKR

SEQ ID NO: 45 - protein, 244 aa, antiFAP-scFv
QVQLVQSGAEVKKPGSSVKVSCKASGGTFSSYAISWVRQAPGQGLEWMGGIIPIFGTANYAQKFQGRVTITADKSTSTAYMELSSLRSEDTAVYYCARDAADRDYWGQGTTVTVSSGGGGSGGGGSGGGGSDIVMTQSPLSLPVTPGEPASISCRSSQSLLHPNGFNHLYWYLQKPGQSPQLLIYVGGNRASGVPDRFSGSGSGTDFTLKISRVEAEDVGVYYCQQRNNKNRTFGQGTKVEIKR

SEQ ID NO: 46 - protein, 247 aa, anti Claudin18.2 scFv
QVQLQESGPGLIKPSQTLSLTCTVSGGSISSGYNWHWIRQPPGKGLEWIGYIHYTGSTNYNPALRSRVTISVDTSKNQFSLKLSSVTAADTAIYYCARIYNGNSFPYWGQGTTVTVSSGGGGSGGGGSGGGGSDIVMTQSPDSLAVSLGERATINCKSSQSLFNSGNQKNYLTWYQQKPGQPPKLLIYWASTRESGVPDRFSGSGSGTDFTLTISSLQAEDVAVYYCQNAYSFPYTFGGGTKLEIKR

SEQ ID NO: 47 - protein, 241 aa, antiCLL1-scFv
EVQLVQSGAEVKKPGASVKVSCKASGYTFNSYYMHWVRQAPGQGLEWMGIFNPGGGSTSYAQKFQGRVTMTRDTSTSTVYMELSSLRSEDTAVYYCARGTTSDAFDIWGQGTMVTVSSGGGGSGGGGSGGGGSDIQMTQSPSSLSASVGDRVTITCRASQSISSYLNWYQQKPGKAPKLLIDVASSLQSGVPSRFSGSGSGTDFTLTISSLQPEDFATYYCQQSYSTPLTFGGGTKVEIKR

SEQ ID NO: 48 - protein, 144 aa, UAS
AAGCTTGATATCGAATTCGGAGCACTGTCCTCCGAACGTCGGAGCACTGTCCTCCGAACGTCGGAGCACTGTCCTCCGAACGTCGGAGCACTGTCCTCCGAACGGAGCATGTCCTCCGAACGTCGGAGCACTGTCCTCCGAACG

SEQ ID NO: 49 - protein, 288 aa, UAS-CMV promoter
AAGCTTGATATCGAATTCGGAGCACTGTCCTCCGAACGTCGGAGCACTGTCCTCCGAACGTCGGAGCACTGTCCTCCGAACGTCGGAGCACTGTCCTCCGAACGGAGCATGTCCTCCGAACGTCGGAGCACTGTCCTCCGAACGACTAGTTAGGCGTGTACGGTGGGAGGCCTATATAAGCAGAGCTCGTTTAGTGAACCGTCAGATCGCCTGGAGACGCCATCCACGCTGTTTTGACCTCCATAGAAGACACCGGGACCGATCCAGCCTCTCGACATTCGTTGGATC

SEQ ID NO: 50 - protein, 545 aa, Amino acid sequence of CD123-synEphrinB2EC
EVQLLESGGGLVQPGGSLRLSCAASGFTFSSYAMSWVRQAPGKGLEWVSAISGSGGSTYYADSVKGRFTISRDNSKNTLYLQMNSLRAEDTAVYYCAKDDSFYGGFDYWGQGTLVTVSSGGGGSGGGGSGGGGSDIQMTQSPSTLSASVGDRVTITCRASQSISSWLAWYQQKPGKAPKLLIYDASSLESGVPSRFSGSGSGTEFTLTISSLQPDDFATYYCQQYSSYKYTFGQGTKVEIKRGQDASSAGSTRNKDPTRRPELEAGTNGRSSTTSPFVKPNPGSSTDGNSAGHSGNNILGSEVALFALMYVAAAAFVLLFFVGCGVLLSRKRRRMKLLSSIEQACDICRLKKLKCSKEKPKCAKCLKNNWECRYSPKTKRSPLTRAHLTEVESRLERLEQLFLLIFPREDLDMILKMDSLQDIKALLTGLFVQDNVNKDAVTDRLASVETDMPLTLRQHRISATSSSEESSNKGQRQLTVSAAAGGSGGSGGSDALDDFDLDMLGSDALDDFDLDMLGSDALDDFDLDMLGSDALDDFDLDMLGS

SEQ ID NO: 51 - protein, 709 aa, Amino acid sequence of GPC3-synJagged2EC
EQKLISEEDLEVQLVQSGAEVKKPGASVKVSCKASGYTFSDYEMHWVRQAPGQGLEWMGAIHPGSGDTAYNQRFKGRVTITADKSTSTAYMELSSLRSEDTAVYYCARFYSYAYWGQGTLVTVSAGGGGSGGGGSGGGGSDIVMTQTPLSLPVTPGEPASISCRSSQSLVHSNGNTYLQWYLQKPGQSPQLLIYKVSNRFSGVPDRFSGSGSGTDFTLKISRVEAEDVGVYYCSQSIYVPYTFGQGTKLEIKREVIGFGRSCWSRGTPFPHGSSWVEDCNSCRCLDGRRDCSKVWCGWKPCLLAGQPEALSAQCPLGQRCLEKAPGQCLRPPCEAWGECGAEEPPSTPCLPRSGHLDNNCARLTLHFNRDHVPQGTTVGAICSGIRSLPATRAVARDRLLVLLCDRASSGASAVEVAVSFSPARDLPDSSLIQGAAHAIVAAITQRGNSSLLLAVTEVKVETVVTGGSSTGLMYVAAAAFVLLFFVGCGVLLSRKRRRMKLLSSIEQACDICRLKKLKCSKEKPKCAKCLKNNWECRYSPKTKRSPLTRAHLTEVESRLERLEQLFLLIFPREDLDMILKMDSLQDIKALLTGLFVQDNVNKDAVTDRLASVETDMPLTLRQHRISATSSSEESSNKGQRQLTVSAAAGGSGGSGGSDALDDFDLDMLGSDALDDFDLDMLGSDALDDFDLDMLGSDALDDFDLDMLGS

SEQ ID NO: 52 - protein, 556 aa, Amino acid sequence of GPC3-EphrinB2EC
EQKLISEEDLEVQLVQSGAEVKKPGASVKVSCKASGYTFSDYEMHWVRQAPGQGLEWMGAIHPGSGDTAYNQRFKGRVTITADKSTSTAYMELSSLRSEDTAVYYCARFYSYAYWGQGTLVTVSAGGGGSGGGGSGGGGSDIVMTQTPLSLPVTPGEPASISCRSSQSLVHSNGNTYLQWYLQKPGQSPQLLIYKVSNRFSGVPDRFSGSGSGTDFTLKISRVEAEDVGVYYCSQSIYVPYTFGQGTKLEIKRGQDASSAGSTRNKDPTRRPELEAGTNGRSSTTSPFVKPNPGSSTDGNSAGHSGNNILGSEVALFALMYVAAAAFVLLFFVGCGVLLSRKRRRMKLLSSIEQACDICRLKKLKCSKEKPKCAKCLKNNWECRYSPKTKRSPLTRAHLTEVESRLERLEQLFLLIFPREDLDMILKMDSLQDIKALLTGLFVQDNVNKDAVTDRLASVETDMPLTLRQHRISATSSSEESSNKGQRQLTVSAAAGGSGGSGGSDALDDFDLDMLGSDALDDFDLDMLGSDALDDFDLDMLGSDALDDFDLDMLGS

SEQ ID NO: 53 - protein, 557 aa, Amino acid sequence of GPC3- synEphrinB2EC-APLP2(TM)
EQKLISEEDLEVQLVQSGAEVKKPGASVKVSCKASGYTFSDYEMHWVRQAPGQGLEWMGAIHPGSGDTAYNQRFKGRVTITADKSTSTAYMELSSLRSEDTAVYYCARFYSYAYWGQGTLVTVSAGGGGSGGGGSGGGGSDIVMTQTPLSLPVTPGEPASISCRSSQSLVHSNGNTYLQWYLQKPGQSPQLLIYKVSNRFSGVPDRFSGSGSGTDFTLKISRVEAEDVGVYYCSQSIYVPYTFGQGTKLEIKRGQDASSAGSTRNKDPTRRPELEAGTNGRSSTTSPFVKPNPGSSTDGNSAGHSGNNILGSEVALFASALIGLLVIAVAIATVIVISLVMLRKRQMKLLSSIEQACDICRLKKLKCSKEKPKCAKCLKNNWECRYSPKTKRSPLTRAHLTEVESRLERLEQLFLLIFPREDLDMILKMDSLQDIKALLTGLFVQDNVNKDAVTDRLASVETDMPLTLRQHRISATSSSEESSNKGQRQLTVSAAAGGSGGSGGSDALDDFDLDMLGSDALDDFDLDMLGSDALDDFDLDMLGSDALDDFDLDMLGS

SEQ ID NO: 54 - protein, 545 aa, Amino acid sequence of GPC3-synEphrinB2EC-del1
EQKLISEEDLEVQLVQSGAEVKKPGASVKVSCKASGYTFSDYEMHWVRQAPGQGLEWMGAIHPGSGDTAYNQRFKGRVTITADKSTSTAYMELSSLRSEDTAVYYCARFYSYAYWGQGTLVTVSAGGGGSGGGGSGGGGSDIVMTQTPLSLPVTPGEPASISCRSSQSLVHSNGNTYLQWYLQKPGQSPQLLIYKVSNRFSGVPDRFSGSGSGTDFTLKISRVEAEDVGVYYCSQSIYVPYTFGQGTKLEIKRGQDATRRPELEAGTNGRSSTTSPFVKPNPGSSTDGNSAGHSGNNILGSEVALFALMYVAAAAFVLLFFVGCGVLLSRKRRRMKLLSSIEQACDICRLKKLKCSKEKPKCAKCLKNNWECRYSPKTKRSPLTRAHLTEVESRLERLEQLFLLIFPREDLDMILKMDSLQDIKALLTGLFVQDNVNKDAVTDRLASVETDMPLTLRQHRISATSSSEESSNKGQRQLTVSAAAGGSGGSGGSDALDDFDLDMLGSDALDDFDLDMLGSDALDDFDLDMLGSDALDDFDLDMLGS

SEQ ID NO: 55 - protein, 543 aa, Amino acid sequence of GPC3-synEphrinB2EC-del2
EQKLISEEDLEVQLVQSGAEVKKPGASVKVSCKASGYTFSDYEMHWVRQAPGQGLEWMGAIHPGSGDTAYNQRFKGRVTITADKSTSTAYMELSSLRSEDTAVYYCARFYSYAYWGQGTLVTVSAGGGGSGGGGSGGGGSDIVMTQTPLSLPVTPGEPASISCRSSQSLVHSNGNTYLQWYLQKPGQSPQLLIYKVSNRFSGVPDRFSGSGSGTDFTLKISRVEAEDVGVYYCSQSIYVPYTFGQGTKLEIKRGQDASSAGSTRNKDPTRRPSPFVKPNPGSSTDGNSAGHSGNNILGSEVALFALMYVAAAAFVLLFFVGCGVLLSRKRRRMKLLSSIEQACDICRLKKLKCSKEKPKCAKCLKNNWECRYSPKTKRSPLTRAHLTEVESRLERLEQLFLLIFPREDLDMILKMDSLQDIKALLTGLFVQDNVNKDAVTDRLASVETDMPLTLRQHRISATSSSEESSNKGQRQLTVSAAAGGSGGSGGSDALDDFDLDMLGSDALDDFDLDMLGSDALDDFDLDMLGSDALDDFDLDMLGS

SEQ ID NO: 56 - protein, 532 aa, Amino acid sequence of GPC3-synEphrinB2EC-del3
EQKLISEEDLEVQLVQSGAEVKKPGASVKVSCKASGYTFSDYEMHWVRQAPGQGLEWMGAIHPGSGDTAYNQRFKGRVTITADKSTSTAYMELSSLRSEDTAVYYCARFYSYAYWGQGTLVTVSAGGGGSGGGGSGGGGSDIVMTQTPLSLPVTPGEPASISCRSSQSLVHSNGNTYLQWYLQKPGQSPQLLIYKVSNRFSGVPDRFSGSGSGTDFTLKISRVEAEDVGVYYCSQSIYVPYTFGQGTKLEIKRGQDASSAGSTRNKDPTRRPELEAGTNGRSSTTSPSEVALFALMYVAAAAFVLLFFVGCGVLLSRKRRRMKLLSSIEQACDICRLKKLKCSKEKPKCAKCLKNNWECRYSPKTKRSPLTRAHLTEVESRLERLEQLFLLIFPREDLDMILKMDSLQDIKALLTGLFVQDNVNKDAVTDRLASVETDMPLTLRQHRISATSSSEESSNKGQRQLTVSAAAGGSGGSGGSDALDDFDLDMLGSDALDDFDLDMLGSDALDDFDLDMLGSDALDDFDLDMLGS

SEQ ID NO: 57 - protein, 517 aa, Amino acid sequence of GPC3-synEphrinB2EC-del23
EQKLISEEDLEVQLVQSGAEVKKPGASVKVSCKASGYTFSDYEMHWVRQAPGQGLEWMGAIHPGSGDTAYNQRFKGRVTITADKSTSTAYMELSSLRSEDTAVYYCARFYSYAYWGQGTLVTVSAGGGGSGGGGSGGGGSDIVMTQTPLSLPVTPGEPASISCRSSQSLVHSNGNTYLQWYLQKPGQSPQLLIYKVSNRFSGVPDRFSGSGSGTDFTLKISRVEAEDVGVYYCSQSIYVPYTFGQGTKLEIKRGQDASSAGSTRNKDPTRRPSEVALFALMYVAAAAFVLLFFVGCGVLLSRKRRRMKLLSSIEQACDICRLKKLKCSKEKPKCAKCLKNNWECRYSPKTKRSPLTRAHLTEVESRLERLEQLFLLIFPREDLDMILKMDSLQDIKALLTGLFVQDNVNKDAVTDRLASVETDMPLTLRQHRISATSSSEESSNKGQRQLTVSAAAGGSGGSGGSDALDDFDLDMLGSDALDDFDLDMLGSDALDDFDLDMLGSDALDDFDLDMLGS

SEQ ID NO: 58 - protein, 540 aa, IL12(including two subunits P35 and P40)
MCHQQLVISWFSLVFLASPLVAIWELKKDVYVVELDWYPDAPGEMVVLTCDTPEEDGITWTLDQSSEVLGSGKTLTIQVKEFGDAGQYTCHKGGEVLSHSLLLLHKKEDGIWSTDILKDQKEPKNKTFLRCEAKNYSGRFTCWWLTTISTDLTFSVKSSRGSSDPQGVTCGAATLSAERVRGDNKEYEYSVECQEDSACPAAEESLPIEVMVDAVHKLKYENYTSSFFIRDIIKPDPPKNLQLKPLKNSRQVEVSWEYPDTWSTPHSYFSLTFCVQVQGKSKREKKDRVFTDKTSATVICRKNASISVRAQDRYYSSSWSEWASVPCSGGGGSGGGGSGGGGSRNLPVATPDPGMFPCLHHSQNLLRAVSNMLQKARQTLEFYPCTSEEIDHEDITKDKTSTVEACLPLELTKNESCLNSRETSFITNGSCLASRKTSFMMALCLSSIYEDLKMYQVEFKTMNAKLLMDPKRQIFLDQNMLAVIDELMQALNFNSETVPQKSSLEEPDFYKTKIKLCILLHAFRIRAVTIDRVMSYLNAS

SEQ ID NO: 59 - DNA, 3921 bp, Nucleic acid of IL12-GPC3-synEphrinB2EC-del3
aagcttgatatcgaattcggagcactgtcctccgaacgtcggagcactgtcctccgaacgtcggagcactgtcctccgaacgtcggagcactgtcctccgaacggagcatgtcctccgaacgtcggagcactgtcctccgaacgactagttaggcgtgtacggtgggaggcctatataagcagagctcgtttagtgaaccgtcagatcgcctggagacgccatccacgctgttttgacctccatagaagacaccgggaccgatccagcctctcgacattcgttggatcatgtgtcaccagcagttggtcatctcttggttttccctggtttttctggcatctcccctcgtggccatatgggaactgaagaaagatgtttatgtcgtagaattggattggtatccggatgcccctggagaaatggtggtcctcacctgtgacacccctgaagaagatggtatcacctggaccttggaccagagcagtgaggtcttaggctctggcaaaaccctgaccatccaagtcaaagagtttggagatgctggccagtacacctgtcacaaaggaggcgaggttctaagccattcgctcctgctgcttcacaaaaaggaagatggaatttggtccactgatattttaaaggaccagaaagaacccaaaaataagacctttctaagatgcgaggccaagaattattctggacgtttcacctgctggtggctgacgacaatcagtactgatttgacattcagtgtcaaaagcagcagaggctcttctgacccccaaggggtgacgtgcggagctgctacactctctgcagagagagtcagaggggacaacaaggagtatgagtactcagtggagtgccaggaggacagtgcctgcccagctgctgaggagagtctgcccattgaggtcatggtggatgccgttcacaagctcaagtatgaaaactacaccagcagcttcttcatcagggacatcatcaaacctgacccacccaagaacttgcagctgaagccattaaagaattctcggcaggtggaggtcagctgggagtaccctgacacctggagtactccacattcctacttctccctgacattctgcgttcaggtccagggcaagagcaagagagaaaagaaagatagagtcttcacggacaagacctcagccacggtcatctgccgcaaaaatgccagcattagcgtgcgggcccaggaccgctactatagctcatcttggagcgaatgggcatctgtgccctgcagtggtggcggtggctcgggcggtggtgggtcgggtggcggcggatctagaaacctccccgtggccactccagacccaggaatgttcccatgccttcaccactcccaaaacctgctgagggccgtcagcaacatgctccagaaggccagacaaactctagaattttacccttgcacttctgaagagattgatcatgaagatatcacaaaagataaaaccagcacagtggaggcctgtttaccattggaattaaccaagaatgagagttgcctaaattccagagagacctctttcataactaatgggagttgcctggcctccagaaagacctcttttatgatggccctgtgccttagtagtatttatgaagacttgaagatgtaccaggtggagttcaagaccatgaatgcaaagcttctgatggatcctaagaggcagatctttctagatcaaaacatgctggcagttattgatgagctgatgcaggccctgaatttcaacagtgagactgtgccacaaaaatcctcccttgaagaaccggatttttataaaactaaaatcaagctctgcatacttcttcatgctttcagaattcgggcagtgactattgatagagtgatgagctatctgaatgcttcctaaacgcgtggctccggtgcccgtcagtgggcagagcgcacatcgcccacagtccccgagaagttggggggaggggtcggcaattgaaccggtgcctagagaaggtggcgcggggtaaactgggaaagtgatgtcgtgtactggctccgcctttttcccgagggtgggggagaaccgtatataagtgcagtagtcgccgtgaacgttctttttcgcaacgggtttgccgccagaacacaggtgtcgtgacgcggatccaggcctaagcttacgcgtgccaccatggcgctccctgtcaccgcactgcttcttccgctggcactgctgctgcacgctgcacggcctgagcaaaaacttatctctgaagaggacctcgaggtgcagctggtgcagagcggcgccgaggtgaagaagcccggcgccagcgtgaaggtgagctgcaaggccagcggctacaccttcagcgactacgagatgcactgggtgcggcaggcccccggccagggcctggagtggatgggcgccatccaccccggcagcggcgacaccgcctacaaccagcggttcaagggccgggtgaccatcaccgccgacaagagcaccagcaccgcctacatggagctgagcagcctgcggagcgaggacaccgccgtgtactactgcgcccggttctacagctacgcctactggggccagggcaccctggtgaccgtgagcgccggtggaggcggttcaggcggaggtggttctggcggtggcggatcggacatcgtgatgacccagacccccctgagcctgcccgtgacccccggcgagcccgccagcatcagctgccggagcagccagagcctggtgcacagcaacggcaacacctacctgcagtggtacctgcagaagcccggccagagcccccagctgctgatctacaaggtgagcaaccggttcagcggcgtgcccgaccggttcagcggcagcggcagcggcaccgacttcaccctgaagatcagccgggtggaggccgaggacgtgggcgtgtactactgcagccagagcatctacgtgccctacaccttcggccagggcaccaagctggagatcaaacgtggacaagatgcaagttctgctggatcaaccaggaataaagatccaacaagacgtccagaactagaagctggtacaaatggaagaagttcgacaacaagtccctttgtaaaaccaaatccaggttctagcacagacggcaacagcgccggacattcggggaacaacatcctcggttccgaagtggccttatttgcactcatgtacgtggcagcggccgccttcgtgctcctgttctttgtgggctgtggggtgctgctgtcccgcaagcgccggcggatgaagctgctgagcagcatcgagcaggcctgtgacatctgccggctgaagaaactgaagtgcagcaaagaaaagcccaagtgcgccaagtgcctgaagaacaactgggagtgccggtacagccccaagaccaagagaagccccctgaccagagcccacctgaccgaggtggaaagccggctggaaagactggaacagctgtttctgctgatcttcccacgcgaggacctggacatgatcctgaagatggacagcctgcaggacatcaaggccctgctgaccggcctgttcgtgcaggacaacgtgaacaaggacgccgtgaccgacagactggccagcgtggaaaccgacatgcccctgaccctgcggcagcacagaatcagcgccaccagcagcagcgaggaaagcagcaacaagggccagcggcagctgacagtgtctgctgctgcaggcggaagcggaggctctggcggatctgatgccctggacgacttcgacctggatatgctgggcagcgacgccctggatgattttgatctggacatgctgggatctgacgctctggacgatttcgatctcgacatgttgggatcagatgcactggatgactttgacctggacatgctcggatca

SEQ ID NO: 60 - protein, 467 aa, GPC3-CAR
EVQLVQSGAEVKKPGASVKVSCKASGYTFSDYEMHWVRQAPGQGLEWMGAIHPGSGDTAYNQRFKGRVTITADKSTSTAYMELSSLRSEDTAVYYCARFYSYAYWGQGTLVTVSAGGGGSGGGGSGGGGSDIVMTQTPLSLPVTPGEPASISCRSSQSLVHSNGNTYLQWYLQKPGQSPQLLIYKVSNRFSGVPDRFSGSGSGTDFTLKISRVEAEDVGVYYCSQSIYVPYTFGQGTKLEIKRTTTPAPRPPTPAPTIASQPLSLRPEACRPAAGGAVHTRGLDFACDIYIWAPLAGTCGVLLLSLVITLYCKRGRKKLLYIFKQPFMRPVQTTQEEDGCSCRFPEEEEGGCELRVKFSRSADAPAYQQGQNQLYNELNLGRREEYDVLDKRRGRDPEMGGKPQRRKNPQEGLYNELQKDKMAEAYSEIGMKGERRRGKGHDGLYQGLSTATKDTYDALHMQALPPR

SEQ ID NO: 61 - protein, 542 aa, Amino acid sequence of EGFRvⅢ-EphrinB2EC
DIQMTQSPSSLSASVGDRVTITCHASQDINVNIGWLQQKPGKAFKGLIYHGKNLEDGVPSRFSGSGSGTDFTLTISSLQPEDFATYYCNQYENIPLTFGQGTKVEIKRGGGGSGGGGSGGGGSDVQLVESGGGLVQPGGSLRLSCAVSGYSITSDYAWNWIRQAPGKGLEWLGYISYRGRTQYNPSLKSRISITRDNSKNTFFLQLNSLRAEDTAVYYCARMGKNWDYWGQGTLVTVSSGQDASSAGSTRNKDPTRRPELEAGTNGRSSTTSPFVKPNPGSSTDGNSAGHSGNNILGSEVALFALMYVAAAAFVLLFFVGCGVLLSRKRRRMKLLSSIEQACDICRLKKLKCSKEKPKCAKCLKNNWECRYSPKTKRSPLTRAHLTEVESRLERLEQLFLLIFPREDLDMILKMDSLQDIKALLTGLFVQDNVNKDAVTDRLASVETDMPLTLRQHRISATSSSEESSNKGQRQLTVSAAAGGSGGSGGSDALDDFDLDMLGSDALDDFDLDMLGSDALDDFDLDMLGSDALDDFDLDMLGS

SEQ ID NO: 62 - protein, 471 aa, Amino acid of IL13Ra2-CAR
EVQLLESGGGLVQPGGSLRLSCAASGFTFRKYAMGWVRQAPGKGLEWVSGISGSVGSTYYADSVKGRFTISRDNSKNTLYLQMNSLRAEDTAVYYCAKVRYGWGAGAFDYWGQGTLVTVSSGGGGSGGGGSGGGGSDIQMTQSPSTLSASVGDRVTITCRASQSISSWLAWYQQKPGKAPKLLIYDASSLESGVPSRFSGSGSGTEFTLTISSLQPDDFATYYCQQYDTYPPITFGQGTKVEIKRTTTPAPRPPTPAPTIASQPLSLRPEACRPAAGGAVHTRGLDFACDFWVLVVVGGVLACYSLLVTVAFIIFWVRSKRSRLLHSDYMNMTPRRPGPTRKHYQPYAPPRDFAAYRSRVKFSRSADAPAYQQGQNQLYNELNLGRREEYDVLDKRRGRDPEMGGKPQRRKNPQEGLYNELQKDKMAEAYSEIGMKGERRRGKGHDGLYQGLSTATKDTYDALHMQALPPR

SEQ ID NO: 63 - DNA, 3735 bp, Nucleic acid of EGFRvⅢ-EphrinB2EC-IL13Ra2-CAR
aagcttgatatcgaattcggagcactgtcctccgaacgtcggagcactgtcctccgaacgtcggagcactgtcctccgaacgtcggagcactgtcctccgaacggagcatgtcctccgaacgtcggagcactgtcctccgaacgactagttaggcgtgtacggtgggaggcctatataagcagagctcgtttagtgaaccgtcagatcgcctggagacgccatccacgctgttttgacctccatagaagacaccgggaccgatccagcctctcgacattcgttggatcatggccttaccagtgaccgccttgctcctgccgctggccttgctgctccacgccgccaggccggaggtgcaattgctggagtctgggggaggcttggtacagcctggggggtccctgagactctcctgtgcagcctccggattcacctttcgcaagtatgccatgggctgggtccgccaggctccagggaaggggctggagtgggtctcaggtattagtggtagtgttggtagcacatactacgcagactccgtgaagggccggttcaccatctccagagacaattccaagaacacgctgtatctgcagatgaacagcctgagagccgaggacacggccgtatattactgtgcgaaagttcgttacggttggggtgcaggtgcattcgactactggggccaaggaaccctggtcaccgtctcgagtggtggaggcggttcaggcggaggtggttctggcggtggcggatcggacatccagatgacccagtctccttccaccctgtctgcatctgtaggagaccgtgtcaccatcacttgccgtgccagtcagagtattagtagctggttggcctggtatcagcagaaaccagggaaagcccctaagctcctgatctatgatgcctccagtttggaaagtggggtcccatcacgtttcagcggcagtggatccgggacagaattcactctcaccatcagcagcttgcagcctgatgattttgcaacttattactgccaacagtacgatacctacccaccaatcacgtttggccagggcaccaaagtcgagatcaagcgtaccacgacgccagcgccgcgaccaccaacaccggcgcccaccatcgcgtcgcagcccctgtccctgcgcccagaggcgtgccggccagcggcggggggcgcagtgcacacgagggggctggacttcgcctgtgatttttgggtgctggtggtggttggtggagtcctggcttgctatagcttgctagtaacagtggcctttattattttctgggtgaggagtaagaggagcaggctcctgcacagtgactacatgaacatgactccccgccgccccgggccaacccgcaagcattaccagccctatgccccaccacgcgacttcgcagcctatcgctccagagtgaagttcagcaggagcgcagacgcccccgcgtaccagcagggccagaaccagctctataacgagctcaatctaggacgaagagaggagtacgatgttttggacaagagacgtggccgggaccctgagatggggggaaagccgcagagaaggaagaaccctcaggaaggcctgtacaatgaactgcagaaagataagatggcggaggcctacagtgagattgggatgaaaggcgagcgccggaggggcaaggggcacgatggcctttaccagggtctcagtacagccaccaaggacacctacgacgcccttcacatgcaggccctgccccctcgctagacgcgtggctccggtgcccgtcagtgggcagagcgcacatcgcccacagtccccgagaagttggggggaggggtcggcaattgaaccggtgcctagagaaggtggcgcggggtaaactgggaaagtgatgtcgtgtactggctccgcctttttcccgagggtgggggagaaccgtatataagtgcagtagtcgccgtgaacgttctttttcgcaacgggtttgccgccagaacacaggtgtcgtgacgcggatccaggcctaagcttacgcgtgccaccatggccttaccagtgaccgccttgctcctgccgctggccttgctgctccacgccgccaggccggatattcagatgacccagagcccgagcagcctgagcgcgagcgtgggcgaccgtgtgaccattacctgccatgcgagccaggatattaacgtgaacattggctggctgcagcagaaaccgggcaaagcgtttaaaggcctgatttatcatggcaaaaacctggaagatggcgtgccgagccgttttagcggcagcggcagcggcaccgattttaccctgaccattagcagcctgcagccggaagattttgcgacctattattgcaatcagtatgaaaatatcccactgacatttggccagggcaccaaagtggaaattaaacgtggtggaggcggttcaggcggaggtggctctggcggtggcggatcggatgtgcagctggtggaaagcggcggcggcctggtgcagccgggcggcagcctgcgtctgagctgcgcggtgagcggctatagcattaccagcgattatgcgtggaactggattcgtcaggcgccgggcaaaggcctggaatggctgggctatattagctatcgtggccgcacccagtataacccgagcctgaaaagccgtattagcattacccgtgataacagcaaaaacacctttttcctgcagctgaacagcctgcgtgcggaagataccgcggtgtattattgcgcgcgcatgggtaagaattgggattactggggccagggcaccctggtgaccgtgagcagcggacaagatgcaagttctgctggatcaaccaggaataaagatccaacaagacgtccagaactagaagctggtacaaatggaagaagttcgacaacaagtccctttgtaaaaccaaatccaggttctagcacagacggcaacagcgccggacattcggggaacaacatcctcggttccgaagtggccttatttgcactcatgtacgtggcagcggccgccttcgtgctcctgttctttgtgggctgtggggtgctgctgtcccgcaagcgccggcggatgaagctgctgagcagcatcgagcaggcctgtgacatctgccggctgaagaaactgaagtgcagcaaagaaaagcccaagtgcgccaagtgcctgaagaacaactgggagtgccggtacagccccaagaccaagagaagccccctgaccagagcccacctgaccgaggtggaaagccggctggaaagactggaacagctgtttctgctgatcttcccacgcgaggacctggacatgatcctgaagatggacagcctgcaggacatcaaggccctgctgaccggcctgttcgtgcaggacaacgtgaacaaggacgccgtgaccgacagactggccagcgtggaaaccgacatgcccctgaccctgcggcagcacagaatcagcgccaccagcagcagcgaggaaagcagcaacaagggccagcggcagctgacagtgtctgctgctgcaggcggaagcggaggctctggcggatctgatgccctggacgacttcgacctggatatgctgggcagcgacgccctggatgattttgatctggacatgctgggatctgacgctctggacgatttcgatctcgacatgttgggatcagatgcactggatgactttgacctggacatgctcggatca

SEQ ID NO: 64 - protein, 467 aa, Amino acid of B7H3-28Z
EVQLLESGGGLVQPGGSLRLSCAASGFTFSSYAMSWVRQAPGKGLEWVSAISGSGGSTYYADSVKGRFTISRDNSKNTLYLQMNSLRAEDTAVYYCAKYRAVTFDYWGQGTLVTVSSGGGGSGGGGSGGGGSDIQMTQSPSTLSASVGDRVTITCRASQSISSWLAWYQQKPGKAPKLLIYDASSLESGVPSRFSGSGSGTEFTLTISSLQPDDFATYYCQQFETQIRWTFGQGTKVEIKRTTTPAPRPPTPAPTIASQPLSLRPEACRPAAGGAVHTRGLDFACDFWVLVVVGGVLACYSLLVTVAFIIFWVRSKRSRLLHSDYMNMTPRRPGPTRKHYQPYAPPRDFAAYRSRVKFSRSADAPAYQQGQNQLYNELNLGRREEYDVLDKRRGRDPEMGGKPQRRKNPQEGLYNELQKDKMAEAYSEIGMKGERRRGKGHDGLYQGLSTATKDTYDALHMQALPPR

SEQ ID NO: 65 - protein, 465 aa, Amino acid of B7H3-BBZ
EVQLLESGGGLVQPGGSLRLSCAASGFTFSSYAMSWVRQAPGKGLEWVSAISGSGGSTYYADSVKGRFTISRDNSKNTLYLQMNSLRAEDTAVYYCAKYRAVTFDYWGQGTLVTVSSGGGGSGGGGSGGGGSDIQMTQSPSTLSASVGDRVTITCRASQSISSWLAWYQQKPGKAPKLLIYDASSLESGVPSRFSGSGSGTEFTLTISSLQPDDFATYYCQQFETQIRWTFGQGTKVEIKRTTTPAPRPPTPAPTIASQPLSLRPEACRPAAGGAVHTRGLDFACDIYIWAPLAGTCGVLLLSLVITLYCKRGRKKLLYIFKQPFMRPVQTTQEEDGCSCRFPEEEEGGCELRVKFSRSADAPAYQQGQNQLYNELNLGRREEYDVLDKRRGRDPEMGGKPQRRKNPQEGLYNELQKDKMAEAYSEIGMKGERRRGKGHDGLYQGLSTATKDTYDALHMQALPPR

SEQ ID NO: 66 - protein, 466 aa, Amino acid of 376.96-28Z
DIVMTQSHKFMSTSIGARVSITCKASQDVRTAVAWYQQKPGQSPKLLIYSASYRYTGVPDRFTGSGSGTDFTFTISSVQAEDLAVYYCQQHYGTPPWTFGGGTKLEIKGGGGSGGGGSGGGGSEVQLVESGGGLVKPGGSLKLSCEASRFTFSSYAMSWVRQTPEKRLEWVAAISGGGRYTYYPDSMKGRFTISRDNAKNFLYLQMSSLRSEDTAMYYCARHYDGYLDYWGQGTTLTVSSTTTPAPRPPTPAPTIASQPLSLRPEACRPAAGGAVHTRGLDFACDFWVLVVVGGVLACYSLLVTVAFIIFWVRSKRSRLLHSDYMNMTPRRPGPTRKHYQPYAPPRDFAAYRSRVKFSRSADAPAYQQGQNQLYNELNLGRREEYDVLDKRRGRDPEMGGKPQRRKNPQEGLYNELQKDKMAEAYSEIGMKGERRRGKGHDGLYQGLSTATKDTYDALHMQALPPR

SEQ ID NO: 67 - protein, 471 aa, Claudin18.2-CAR
QVQLQESGPGLIKPSQTLSLTCTVSGGSISSGYNWHWIRQPPGKGLEWIGYIHYTGSTNYNPALRSRVTISVDTSKNQFSLKLSSVTAADTAIYYCARIYNGNSFPYWGQGTTVTVSSGGGGSGGGGSGGGGSDIVMTQSPDSLAVSLGERATINCKSSQSLFNSGNQKNYLTWYQQKPGQPPKLLIYWASTRESGVPDRFSGSGSGTDFTLTISSLQAEDVAVYYCQNAYSFPYTFGGGTKLEIKRTTTPAPRPPTPAPTIASQPLSLRPEACRPAAGGAVHTRGLDFACDIYIWAPLAGTCGVLLLSLVITLYCKRGRKKLLYIFKQPFMRPVQTTQEEDGCSCRFPEEEEGGCELRVKFSRSADAPAYQQGQNQLYNELNLGRREEYDVLDKRRGRDPEMGGKPQRRKNPQEGLYNELQKDKMAEAYSEIGMKGERRRGKGHDGLYQGLSTATKDTYDALHMQALPPR

SEQ ID NO: 68 - DNA, 3766 bp, Mesothelin-synEphrinB2EC- Claudin18.2-CAR
aagcttgatatcgaattcggagcactgtcctccgaacgtcggagcactgtcctccgaacgtcggagcactgtcctccgaacgtcggagcactgtcctccgaacggagcatgtcctccgaacgtcggagcactgtcctccgaacgactagttaggcgtgtacggtgggaggcctatataagcagagctcgtttagtgaaccgtcagatcgcctggagacgccatccacgctgttttgacctccatagaagacaccgggaccgatccagcctctcgacattcgttggatcatggccttaccagtgaccgccttgctcctgccgctggccttgctgctccacgccgccaggccgcaggtgcagctgcaggagagcggccccggcctgatcaagcccagccagaccctgagcctgacctgcaccgtgagcggcggcagcatcagcagcggctacaactggcactggatccggcagccccccggcaagggcctggagtggatcggctacatccactacaccggcagcaccaactacaaccccgccctgcggagccgggtgaccatcagcgtggacaccagcaagaaccagttcagcctgaagctgagcagcgtgaccgccgccgacaccgccatctactactgcgcccggatctacaacggcaacagcttcccctactggggccagggcaccaccgtgaccgtgagcagcggtggaggcggttcaggcggaggtggttctggcggtggcggatcggacatcgtgatgacccagagccccgacagcctggccgtgagcctgggcgagcgggccaccatcaactgcaagagcagccagagcctgttcaacagcggcaaccagaagaactacctgacctggtaccagcagaagcccggccagccccccaagctgctgatctactgggccagcacccgggagagcggcgtgcccgaccggttcagcggcagcggcagcggcaccgacttcaccctgaccatcagcagcctgcaggccgaggacgtggccgtgtactactgccagaacgcctacagcttcccctacaccttcggcggcggcaccaagctggagatcaagcggaccacgacgccagcgccgcgaccaccaacaccggcgcccaccatcgcgtcgcagcccctgtccctgcgcccagaggcgtgccggccagcggcggggggcgcagtgcacacgagggggctggacttcgcctgtgatatctacatctgggcgcccttggccgggacttgtggggtccttctcctgtcactggttatcaccctttactgcaaacggggcagaaagaaactcctgtatatattcaaacaaccatttatgagaccagtacaaactactcaagaggaagatggctgtagctgccgatttccagaagaagaagaaggaggatgtgaactgagagtgaagttcagcaggagcgcagacgcccccgcgtaccagcagggccagaaccagctctataacgagctcaatctaggacgaagagaggagtacgatgttttggacaagagacgtggccgggaccctgagatggggggaaagccgcagagaaggaagaaccctcaggaaggcctgtacaatgaactgcagaaagataagatggcggaggcctacagtgagattgggatgaaaggcgagcgccggaggggcaaggggcacgatggcctttaccagggtctcagtacagccaccaaggacacctacgacgcccttcacatgcaggccctgccccctcgctagtaagctagccgatggctccggtgcccgtcagtgggcagagcgcacatcgcccacagtccccgagaagttggggggaggggtcggcaattgaaccggtgcctagagaaggtggcgcggggtaaactgggaaagtgatgtcgtgtactggctccgcctttttcccgagggtgggggagaaccgtatataagtgcagtagtcgccgtgaacgttctttttcgcaacgggtttgccgccagaacacaggtgtcgtgacgcggatccaggcctaagcttacgcgtgccaccatggcgctccctgtcaccgcactgcttcttccgctggcactgctgctgcacgctgcacggcctcagatgcagctagtgcagtctggggctgaggtgaagaagcctggggcctcagtgaaggtttcctgcaaggcatctggatacaccttcaccagctactatatgcactgggtgcgacaggcccctggacaagggcttgagtggatgggaataatcaaccctagtggtggtagcacaagctacgcacagaagttccagggcagagtcaccatgaccagggacacgtccacgagcacagtctacatggagctgagcagcctgagatctgaggacacggccgtgtattactgtgcgagtagtcggagtgggactacggtggtaaatcatgatgcttttgatatctgggggaaagggaccacggtcaccgtctcgagtggtggaggcggttcaggcggaggtggttctggcggtggcggatcggacatccagttgacccagtctccatcctccctgtctgcgtctgtaggagacagagtcaccatcacttgccgggcaagccaggtcattagccgtgctttagcctggtatcaacaaacaccagggaaacctcctaaactcctgatctatgatgcctccaatttgcagagtggggtcccatcaaggttcagcggcagtggatctgggacagatttcactctcaccatcagccgcctgcagcctgaagattttgcaacttattactgtcaacagtttaatagttaccctctcactttcggcggagggaccaagctggagatcaaacgtggacaagatgcaagttctgctggatcaaccaggaataaagatccaacaagacgtccagaactagaagctggtacaaatggaagaagttcgacaacaagtccctttgtaaaaccaaatccaggttctagcacagacggcaacagcgccggacattcggggaacaacatcctcggttccgaagtggccttatttgcactcatgtacgtggcagcggccgccttcgtgctcctgttctttgtgggctgtggggtgctgctgtcccgcaagcgccggcggatgaagctgctgagcagcatcgagcaggcctgtgacatctgccggctgaagaaactgaagtgcagcaaagaaaagcccaagtgcgccaagtgcctgaagaacaactgggagtgccggtacagccccaagaccaagagaagccccctgaccagagcccacctgaccgaggtggaaagccggctggaaagactggaacagctgtttctgctgatcttcccacgcgaggacctggacatgatcctgaagatggacagcctgcaggacatcaaggccctgctgaccggcctgttcgtgcaggacaacgtgaacaaggacgccgtgaccgacagactggccagcgtggaaaccgacatgcccctgaccctgcggcagcacagaatcagcgccaccagcagcagcgaggaaagcagcaacaagggccagcggcagctgacagtgtctgctgctgcaggcggaagcggaggctctggcggatctgatgccctggacgacttcgacctggatatgctgggcagcgacgccctggatgattttgatctggacatgctgggatctgacgctctggacgatttcgatctcgacatgttgggatcagatgcactggatgactttgacctggacatgctcggatca

SEQ ID NO: 69 - DNA, 4354 bp, Mesothelin-synEphrinB2EC- Claudin18.2-CAR-IL7
aagcttgatatcgaattcggagcactgtcctccgaacgtcggagcactgtcctccgaacgtcggagcactgtcctccgaacgtcggagcactgtcctccgaacggagcatgtcctccgaacgtcggagcactgtcctccgaacgactagttaggcgtgtacggtgggaggcctatataagcagagctcgtttagtgaaccgtcagatcgcctggagacgccatccacgctgttttgacctccatagaagacaccgggaccgatccagcctctcgacattcgttggatcatggccttaccagtgaccgccttgctcctgccgctggccttgctgctccacgccgccaggccgcaggtgcagctgcaggagagcggccccggcctgatcaagcccagccagaccctgagcctgacctgcaccgtgagcggcggcagcatcagcagcggctacaactggcactggatccggcagccccccggcaagggcctggagtggatcggctacatccactacaccggcagcaccaactacaaccccgccctgcggagccgggtgaccatcagcgtggacaccagcaagaaccagttcagcctgaagctgagcagcgtgaccgccgccgacaccgccatctactactgcgcccggatctacaacggcaacagcttcccctactggggccagggcaccaccgtgaccgtgagcagcggtggaggcggttcaggcggaggtggttctggcggtggcggatcggacatcgtgatgacccagagccccgacagcctggccgtgagcctgggcgagcgggccaccatcaactgcaagagcagccagagcctgttcaacagcggcaaccagaagaactacctgacctggtaccagcagaagcccggccagccccccaagctgctgatctactgggccagcacccgggagagcggcgtgcccgaccggttcagcggcagcggcagcggcaccgacttcaccctgaccatcagcagcctgcaggccgaggacgtggccgtgtactactgccagaacgcctacagcttcccctacaccttcggcggcggcaccaagctggagatcaagcggaccacgacgccagcgccgcgaccaccaacaccggcgcccaccatcgcgtcgcagcccctgtccctgcgcccagaggcgtgccggccagcggcggggggcgcagtgcacacgagggggctggacttcgcctgtgatatctacatctgggcgcccttggccgggacttgtggggtccttctcctgtcactggttatcaccctttactgcaaacggggcagaaagaaactcctgtatatattcaaacaaccatttatgagaccagtacaaactactcaagaggaagatggctgtagctgccgatttccagaagaagaagaaggaggatgtgaactgagagtgaagttcagcaggagcgcagacgcccccgcgtaccagcagggccagaaccagctctataacgagctcaatctaggacgaagagaggagtacgatgttttggacaagagacgtggccgggaccctgagatggggggaaagccgcagagaaggaagaaccctcaggaaggcctgtacaatgaactgcagaaagataagatggcggaggcctacagtgagattgggatgaaaggcgagcgccggaggggcaaggggcacgatggcctttaccagggtctcagtacagccaccaaggacacctacgacgcccttcacatgcaggccctgccccctcgcgctactaacttcagcctgctgaagcaggctggagacgtggaggagaaccctggacctatgttccatgtttcttttaggtatatctttggacttcctcccctgatccttgttctgttgccagtagcatcatctgattgtgatattgaaggtaaagatggcaaacaatatgagagtgttctaatggtcagcatcgatcaattattggacagcatgaaagaaattggtagcaattgcctgaataatgaatttaacttttttaaaagacatatctgtgatgctaataaggaaggtatgtttttattccgtgctgctcgcaagttgaggcaatttcttaaaatgaatagcactggtgattttgatctccacttattaaaagtttcagaaggcacaacaatactgttgaactgcactggccaggttaaaggaagaaaaccagctgccctgggtgaagcccaaccaacaaagagtttggaagaaaataaatctttaaaggaacagaaaaaactgaatgacttgtgtttcctaaagagactattacaagagataaaaacttgttggaataaaattttgatgggcactaaagaacactagtaagctagccgatggctccggtgcccgtcagtgggcagagcgcacatcgcccacagtccccgagaagttggggggaggggtcggcaattgaaccggtgcctagagaaggtggcgcggggtaaactgggaaagtgatgtcgtgtactggctccgcctttttcccgagggtgggggagaaccgtatataagtgcagtagtcgccgtgaacgttctttttcgcaacgggtttgccgccagaacacaggtgtcgtgacgcggatccaggcctaagcttacgcgtgccaccatggcgctccctgtcaccgcactgcttcttccgctggcactgctgctgcacgctgcacggcctcagatgcagctagtgcagtctggggctgaggtgaagaagcctggggcctcagtgaaggtttcctgcaaggcatctggatacaccttcaccagctactatatgcactgggtgcgacaggcccctggacaagggcttgagtggatgggaataatcaaccctagtggtggtagcacaagctacgcacagaagttccagggcagagtcaccatgaccagggacacgtccacgagcacagtctacatggagctgagcagcctgagatctgaggacacggccgtgtattactgtgcgagtagtcggagtgggactacggtggtaaatcatgatgcttttgatatctgggggaaagggaccacggtcaccgtctcgagtggtggaggcggttcaggcggaggtggttctggcggtggcggatcggacatccagttgacccagtctccatcctccctgtctgcgtctgtaggagacagagtcaccatcacttgccgggcaagccaggtcattagccgtgctttagcctggtatcaacaaacaccagggaaacctcctaaactcctgatctatgatgcctccaatttgcagagtggggtcccatcaaggttcagcggcagtggatctgggacagatttcactctcaccatcagccgcctgcagcctgaagattttgcaacttattactgtcaacagtttaatagttaccctctcactttcggcggagggaccaagctggagatcaaacgtggacaagatgcaagttctgctggatcaaccaggaataaagatccaacaagacgtccagaactagaagctggtacaaatggaagaagttcgacaacaagtccctttgtaaaaccaaatccaggttctagcacagacggcaacagcgccggacattcggggaacaacatcctcggttccgaagtggccttatttgcactcatgtacgtggcagcggccgccttcgtgctcctgttctttgtgggctgtggggtgctgctgtcccgcaagcgccggcggatgaagctgctgagcagcatcgagcaggcctgtgacatctgccggctgaagaaactgaagtgcagcaaagaaaagcccaagtgcgccaagtgcctgaagaacaactgggagtgccggtacagccccaagaccaagagaagccccctgaccagagcccacctgaccgaggtggaaagccggctggaaagactggaacagctgtttctgctgatcttcccacgcgaggacctggacatgatcctgaagatggacagcctgcaggacatcaaggccctgctgaccggcctgttcgtgcaggacaacgtgaacaaggacgccgtgaccgacagactggccagcgtggaaaccgacatgcccctgaccctgcggcagcacagaatcagcgccaccagcagcagcgaggaaagcagcaacaagggccagcggcagctgacagtgtctgctgctgcaggcggaagcggaggctctggcggatctgatgccctggacgacttcgacctggatatgctgggcagcgacgccctggatgattttgatctggacatgctgggatctgacgctctggacgatttcgatctcgacatgttgggatcagatgcactggatgactttgacctggacatgctcggatca

SEQ ID NO: 70 - DNA, 4810 bp, Mesothelin-synEphrinB2EC- Claudin18.2-CAR-IL7-CCL21
aagcttgatatcgaattcggagcactgtcctccgaacgtcggagcactgtcctccgaacgtcggagcactgtcctccgaacgtcggagcactgtcctccgaacggagcatgtcctccgaacgtcggagcactgtcctccgaacgactagttaggcgtgtacggtgggaggcctatataagcagagctcgtttagtgaaccgtcagatcgcctggagacgccatccacgctgttttgacctccatagaagacaccgggaccgatccagcctctcgacattcgttggatcatggccttaccagtgaccgccttgctcctgccgctggccttgctgctccacgccgccaggccgcaggtgcagctgcaggagagcggccccggcctgatcaagcccagccagaccctgagcctgacctgcaccgtgagcggcggcagcatcagcagcggctacaactggcactggatccggcagccccccggcaagggcctggagtggatcggctacatccactacaccggcagcaccaactacaaccccgccctgcggagccgggtgaccatcagcgtggacaccagcaagaaccagttcagcctgaagctgagcagcgtgaccgccgccgacaccgccatctactactgcgcccggatctacaacggcaacagcttcccctactggggccagggcaccaccgtgaccgtgagcagcggtggaggcggttcaggcggaggtggttctggcggtggcggatcggacatcgtgatgacccagagccccgacagcctggccgtgagcctgggcgagcgggccaccatcaactgcaagagcagccagagcctgttcaacagcggcaaccagaagaactacctgacctggtaccagcagaagcccggccagccccccaagctgctgatctactgggccagcacccgggagagcggcgtgcccgaccggttcagcggcagcggcagcggcaccgacttcaccctgaccatcagcagcctgcaggccgaggacgtggccgtgtactactgccagaacgcctacagcttcccctacaccttcggcggcggcaccaagctggagatcaagcggaccacgacgccagcgccgcgaccaccaacaccggcgcccaccatcgcgtcgcagcccctgtccctgcgcccagaggcgtgccggccagcggcggggggcgcagtgcacacgagggggctggacttcgcctgtgatatctacatctgggcgcccttggccgggacttgtggggtccttctcctgtcactggttatcaccctttactgcaaacggggcagaaagaaactcctgtatatattcaaacaaccatttatgagaccagtacaaactactcaagaggaagatggctgtagctgccgatttccagaagaagaagaaggaggatgtgaactgagagtgaagttcagcaggagcgcagacgcccccgcgtaccagcagggccagaaccagctctataacgagctcaatctaggacgaagagaggagtacgatgttttggacaagagacgtggccgggaccctgagatggggggaaagccgcagagaaggaagaaccctcaggaaggcctgtacaatgaactgcagaaagataagatggcggaggcctacagtgagattgggatgaaaggcgagcgccggaggggcaaggggcacgatggcctttaccagggtctcagtacagccaccaaggacacctacgacgcccttcacatgcaggccctgccccctcgcgctactaacttcagcctgctgaagcaggctggagacgtggaggagaaccctggacctatgttccatgtttcttttaggtatatctttggacttcctcccctgatccttgttctgttgccagtagcatcatctgattgtgatattgaaggtaaagatggcaaacaatatgagagtgttctaatggtcagcatcgatcaattattggacagcatgaaagaaattggtagcaattgcctgaataatgaatttaacttttttaaaagacatatctgtgatgctaataaggaaggtatgtttttattccgtgctgctcgcaagttgaggcaatttcttaaaatgaatagcactggtgattttgatctccacttattaaaagtttcagaaggcacaacaatactgttgaactgcactggccaggttaaaggaagaaaaccagctgccctgggtgaagcccaaccaacaaagagtttggaagaaaataaatctttaaaggaacagaaaaaactgaatgacttgtgtttcctaaagagactattacaagagataaaaacttgttggaataaaattttgatgggcactaaagaacacgagggcagaggaagtctgctaacatgcggtgacgtcgaggagaatcctggacctatggctcagtcactggctctgagcctccttatcctggttctggcctttggcatccccaggacccaaggcagtgatggaggggctcaggactgttgcctcaagtacagccaaaggaagattcccgccaaggttgtccgcagctaccggaagcaggaaccaagcttaggctgctccatcccagctatcctgttcttgccccgcaagcgctctcaggcagagctatgtgcagacccaaaggagctctgggtgcagcagctgatgcagcatctggacaagacaccatccccacagaaaccagcccagggctgcaggaaggacaggggggcctccaagactggcaagaaaggaaagggctccaaaggctgcaagaggactgagcggtcacagacccctaaagggccatagtaagctagccgatggctccggtgcccgtcagtgggcagagcgcacatcgcccacagtccccgagaagttggggggaggggtcggcaattgaaccggtgcctagagaaggtggcgcggggtaaactgggaaagtgatgtcgtgtactggctccgcctttttcccgagggtgggggagaaccgtatataagtgcagtagtcgccgtgaacgttctttttcgcaacgggtttgccgccagaacacaggtgtcgtgacgcggatccaggcctaagcttacgcgtgccaccatggcgctccctgtcaccgcactgcttcttccgctggcactgctgctgcacgctgcacggcctcagatgcagctagtgcagtctggggctgaggtgaagaagcctggggcctcagtgaaggtttcctgcaaggcatctggatacaccttcaccagctactatatgcactgggtgcgacaggcccctggacaagggcttgagtggatgggaataatcaaccctagtggtggtagcacaagctacgcacagaagttccagggcagagtcaccatgaccagggacacgtccacgagcacagtctacatggagctgagcagcctgagatctgaggacacggccgtgtattactgtgcgagtagtcggagtgggactacggtggtaaatcatgatgcttttgatatctgggggaaagggaccacggtcaccgtctcgagtggtggaggcggttcaggcggaggtggttctggcggtggcggatcggacatccagttgacccagtctccatcctccctgtctgcgtctgtaggagacagagtcaccatcacttgccgggcaagccaggtcattagccgtgctttagcctggtatcaacaaacaccagggaaacctcctaaactcctgatctatgatgcctccaatttgcagagtggggtcccatcaaggttcagcggcagtggatctgggacagatttcactctcaccatcagccgcctgcagcctgaagattttgcaacttattactgtcaacagtttaatagttaccctctcactttcggcggagggaccaagctggagatcaaacgtggacaagatgcaagttctgctggatcaaccaggaataaagatccaacaagacgtccagaactagaagctggtacaaatggaagaagttcgacaacaagtccctttgtaaaaccaaatccaggttctagcacagacggcaacagcgccggacattcggggaacaacatcctcggttccgaagtggccttatttgcactcatgtacgtggcagcggccgccttcgtgctcctgttctttgtgggctgtggggtgctgctgtcccgcaagcgccggcggatgaagctgctgagcagcatcgagcaggcctgtgacatctgccggctgaagaaactgaagtgcagcaaagaaaagcccaagtgcgccaagtgcctgaagaacaactgggagtgccggtacagccccaagaccaagagaagccccctgaccagagcccacctgaccgaggtggaaagccggctggaaagactggaacagctgtttctgctgatcttcccacgcgaggacctggacatgatcctgaagatggacagcctgcaggacatcaaggccctgctgaccggcctgttcgtgcaggacaacgtgaacaaggacgccgtgaccgacagactggccagcgtggaaaccgacatgcccctgaccctgcggcagcacagaatcagcgccaccagcagcagcgaggaaagcagcaacaagggccagcggcagctgacagtgtctgctgctgcaggcggaagcggaggctctggcggatctgatgccctggacgacttcgacctggatatgctgggcagcgacgccctggatgattttgatctggacatgctgggatctgacgctctggacgatttcgatctcgacatgttgggatcagatgcactggatgactttgacctggacatgctcggatca

SEQ ID NO: 71 - DNA, 3757 bp, FAP-synEphrinB2EC-Claudin18.2-CAR
aagcttgatatcgaattcggagcactgtcctccgaacgtcggagcactgtcctccgaacgtcggagcactgtcctccgaacgtcggagcactgtcctccgaacggagcatgtcctccgaacgtcggagcactgtcctccgaacgactagttaggcgtgtacggtgggaggcctatataagcagagctcgtttagtgaaccgtcagatcgcctggagacgccatccacgctgttttgacctccatagaagacaccgggaccgatccagcctctcgacattcgttggatcatggccttaccagtgaccgccttgctcctgccgctggccttgctgctccacgccgccaggccgcaggtgcagctgcaggagagcggccccggcctgatcaagcccagccagaccctgagcctgacctgcaccgtgagcggcggcagcatcagcagcggctacaactggcactggatccggcagccccccggcaagggcctggagtggatcggctacatccactacaccggcagcaccaactacaaccccgccctgcggagccgggtgaccatcagcgtggacaccagcaagaaccagttcagcctgaagctgagcagcgtgaccgccgccgacaccgccatctactactgcgcccggatctacaacggcaacagcttcccctactggggccagggcaccaccgtgaccgtgagcagcggtggaggcggttcaggcggaggtggttctggcggtggcggatcggacatcgtgatgacccagagccccgacagcctggccgtgagcctgggcgagcgggccaccatcaactgcaagagcagccagagcctgttcaacagcggcaaccagaagaactacctgacctggtaccagcagaagcccggccagccccccaagctgctgatctactgggccagcacccgggagagcggcgtgcccgaccggttcagcggcagcggcagcggcaccgacttcaccctgaccatcagcagcctgcaggccgaggacgtggccgtgtactactgccagaacgcctacagcttcccctacaccttcggcggcggcaccaagctggagatcaagcggaccacgacgccagcgccgcgaccaccaacaccggcgcccaccatcgcgtcgcagcccctgtccctgcgcccagaggcgtgccggccagcggcggggggcgcagtgcacacgagggggctggacttcgcctgtgatatctacatctgggcgcccttggccgggacttgtggggtccttctcctgtcactggttatcaccctttactgcaaacggggcagaaagaaactcctgtatatattcaaacaaccatttatgagaccagtacaaactactcaagaggaagatggctgtagctgccgatttccagaagaagaagaaggaggatgtgaactgagagtgaagttcagcaggagcgcagacgcccccgcgtaccagcagggccagaaccagctctataacgagctcaatctaggacgaagagaggagtacgatgttttggacaagagacgtggccgggaccctgagatggggggaaagccgcagagaaggaagaaccctcaggaaggcctgtacaatgaactgcagaaagataagatggcggaggcctacagtgagattgggatgaaaggcgagcgccggaggggcaaggggcacgatggcctttaccagggtctcagtacagccaccaaggacacctacgacgcccttcacatgcaggccctgccccctcgctagtaagctagccgatggctccggtgcccgtcagtgggcagagcgcacatcgcccacagtccccgagaagttggggggaggggtcggcaattgaaccggtgcctagagaaggtggcgcggggtaaactgggaaagtgatgtcgtgtactggctccgcctttttcccgagggtgggggagaaccgtatataagtgcagtagtcgccgtgaacgttctttttcgcaacgggtttgccgccagaacacaggtgtcgtgacgcggatccaggcctaagcttacgcgtgccaccatggcgctccctgtcaccgcactgcttcttccgctggcactgctgctgcacgctgcacggcctcaggtgcaattggtgcagtctggggctgaggtgaagaagcctgggtcctcggtgaaggtctcctgcaaggcctccggaggcacattcagcagctacgctataagctgggtgcgacaggcccctggacaagggctcgagtggatgggagggatcatccctatctttggtacagcaaactacgcacagaagttccagggcagggtcaccattactgcagacaaatccacgagcacagcctacatggagctgagcagcctgagatctgaggacaccgccgtgtattactgtgcgagagatgctgctgatagggactactggggccaagggaccaccgtgaccgtctcctcaggtggaggcggttcaggcggaggtggttctggcggtggcggatcggatattgttatgactcaatctccactgtctctgccggtgactccaggcgaaccggcgagcatttcttgccgttccagccagtctctgcttcaccccaacggcttcaaccatctctattggtacctgcaaaaaccgggtcagagccctcagctgctgatctacgtggggggtaaccgcgcttccggtgtaccggaccgtttcagcggctctggatccggcaccgatttcacgttgaaaatcagccgtgttgaagcagaagacgtgggcgtttattactgtcagcagcgtaataataagaatcgtacttttggtcaaggcaccaaggtcgaaattaaacgtggacaagatgcaagttctgctggatcaaccaggaataaagatccaacaagacgtccagaactagaagctggtacaaatggaagaagttcgacaacaagtccctttgtaaaaccaaatccaggttctagcacagacggcaacagcgccggacattcggggaacaacatcctcggttccgaagtggccttatttgcactcatgtacgtggcagcggccgccttcgtgctcctgttctttgtgggctgtggggtgctgctgtcccgcaagcgccggcggatgaagctgctgagcagcatcgagcaggcctgtgacatctgccggctgaagaaactgaagtgcagcaaagaaaagcccaagtgcgccaagtgcctgaagaacaactgggagtgccggtacagccccaagaccaagagaagccccctgaccagagcccacctgaccgaggtggaaagccggctggaaagactggaacagctgtttctgctgatcttcccacgcgaggacctggacatgatcctgaagatggacagcctgcaggacatcaaggccctgctgaccggcctgttcgtgcaggacaacgtgaacaaggacgccgtgaccgacagactggccagcgtggaaaccgacatgcccctgaccctgcggcagcacagaatcagcgccaccagcagcagcgaggaaagcagcaacaagggccagcggcagctgacagtgtctgctgctgcaggcggaagcggaggctctggcggatctgatgccctggacgacttcgacctggatatgctgggcagcgacgccctggatgattttgatctggacatgctgggatctgacgctctggacgatttcgatctcgacatgttgggatcagatgcactggatgactttgacctggacatgctcggatca

SEQ ID NO: 72 - DNA, 3782 bp, Claudin18.2-synEphrinB2EC-Mesothelin-CAR
aagcttgatatcgaattcggagcactgtcctccgaacgtcggagcactgtcctccgaacgtcggagcactgtcctccgaacgtcggagcactgtcctccgaacggagcatgtcctccgaacgtcggagcactgtcctccgaacgactagttaggcgtgtacggtgggaggcctatataagcagagctcgtttagtgaaccgtcagatcgcctggagacgccatccacgctgttttgacctccatagaagacaccgggaccgatccagcctctcgacattcgttggatcatggccttaccagtgaccgccttgctcctgccgctggccttgctgctccacgccgccaggccgcagatgcagctagtgcagtctggggctgaggtgaagaagcctggggcctcagtgaaggtttcctgcaaggcatctggatacaccttcaccagctactatatgcactgggtgcgacaggcccctggacaagggcttgagtggatgggaataatcaaccctagtggtggtagcacaagctacgcacagaagttccagggcagagtcaccatgaccagggacacgtccacgagcacagtctacatggagctgagcagcctgagatctgaggacacggccgtgtattactgtgcgagtagtcggagtgggactacggtggtaaatcatgatgcttttgatatctgggggaaagggaccacggtcaccgtctcgagtggtggaggcggttcaggcggaggtggttctggcggtggcggatcggacatccagttgacccagtctccatcctccctgtctgcgtctgtaggagacagagtcaccatcacttgccgggcaagccaggtcattagccgtgctttagcctggtatcaacaaacaccagggaaacctcctaaactcctgatctatgatgcctccaatttgcagagtggggtcccatcaaggttcagcggcagtggatctgggacagatttcactctcaccatcagccgcctgcagcctgaagattttgcaacttattactgtcaacagtttaatagttaccctctcactttcggcggagggaccaagctggagatcaaacgtaccacgacgccagcgccgcgaccaccaacaccggcgcccaccatcgcgtcgcagcccctgtccctgcgcccagaggcgtgccggccagcggcggggggcgcagtgcacacgagggggctggacttcgcctgtgatatctacatctgggcgcccttggccgggacttgtggggtccttctcctgtcactggttatcaccctttactgcaaacggggcagaaagaaactcctgtatatattcaaacaaccatttatgagaccagtacaaactactcaagaggaagatggctgtagctgccgatttccagaagaagaagaaggaggatgtgaactgagagtgaagttcagcaggagcgcagacgcccccgcgtaccagcagggccagaaccagctctataacgagctcaatctaggacgaagagaggagtacgatgttttggacaagagacgtggccgggaccctgagatggggggaaagccgcagagaaggaagaaccctcaggaaggcctgtacaatgaactgcagaaagataagatggcggaggcctacagtgagattgggatgaaaggcgagcgccggaggggcaaggggcacgatggcctttaccagggtctcagtacagccaccaaggacacctacgacgcccttcacatgcaggccctgccccctcgctagtaagctagccgatggctccggtgcccgtcagtgggcagagcgcacatcgcccacagtccccgagaagttggggggaggggtcggcaattgaaccggtgcctagagaaggtggcgcggggtaaactgggaaagtgatgtcgtgtactggctccgcctttttcccgagggtgggggagaaccgtatataagtgcagtagtcgccgtgaacgttctttttcgcaacgggtttgccgccagaacacaggtgtcgtgacgcggatccaggcctaagcttacgcgtcctagcgctaccggtcgccaccatggccttaccagtgaccgccttgctcctgccgctggccttgctgctccacgccgccaggccgcaggtgcagctgcaggagagcggccccggcctgatcaagcccagccagaccctgagcctgacctgcaccgtgagcggcggcagcatcagcagcggctacaactggcactggatccggcagccccccggcaagggcctggagtggatcggctacatccactacaccggcagcaccaactacaaccccgccctgcggagccgggtgaccatcagcgtggacaccagcaagaaccagttcagcctgaagctgagcagcgtgaccgccgccgacaccgccatctactactgcgcccggatctacaacggcaacagcttcccctactggggccagggcaccaccgtgaccgtgagcagcggtggaggcggttcaggcggaggtggttctggcggtggcggatcggacatcgtgatgacccagagccccgacagcctggccgtgagcctgggcgagcgggccaccatcaactgcaagagcagccagagcctgttcaacagcggcaaccagaagaactacctgacctggtaccagcagaagcccggccagccccccaagctgctgatctactgggccagcacccgggagagcggcgtgcccgaccggttcagcggcagcggcagcggcaccgacttcaccctgaccatcagcagcctgcaggccgaggacgtggccgtgtactactgccagaacgcctacagcttcccctacaccttcggcggcggcaccaagctggagatcaagcggggacaagatgcaagttctgctggatcaaccaggaataaagatccaacaagacgtccagaactagaagctggtacaaatggaagaagttcgacaacaagtccctttgtaaaaccaaatccaggttctagcacagacggcaacagcgccggacattcggggaacaacatcctcggttccgaagtggccttatttgcactcatgtacgtggcagcggccgccttcgtgctcctgttctttgtgggctgtggggtgctgctgtcccgcaagcgccggcggatgaagctgctgagcagcatcgagcaggcctgtgacatctgccggctgaagaaactgaagtgcagcaaagaaaagcccaagtgcgccaagtgcctgaagaacaactgggagtgccggtacagccccaagaccaagagaagccccctgaccagagcccacctgaccgaggtggaaagccggctggaaagactggaacagctgtttctgctgatcttcccacgcgaggacctggacatgatcctgaagatggacagcctgcaggacatcaaggccctgctgaccggcctgttcgtgcaggacaacgtgaacaaggacgccgtgaccgacagactggccagcgtggaaaccgacatgcccctgaccctgcggcagcacagaatcagcgccaccagcagcagcgaggaaagcagcaacaagggccagcggcagctgacagtgtctgctgctgcaggcggaagcggaggctctggcggatctgatgccctggacgacttcgacctggatatgctgggcagcgacgccctggatgattttgatctggacatgctgggatctgacgctctggacgatttcgatctcgacatgttgggatcagatgcactggatgactttgacctggacatgctcggatca

SEQ ID NO: 73 - protein, 544 aa, Amino acid sequence of CLL1-synEphrinB2EC
EVQLVQSGAEVKKPGASVKVSCKASGYTFNSYYMHWVRQAPGQGLEWMGIFNPGGGSTSYAQKFQGRVTMTRDTSTSTVYMELSSLRSEDTAVYYCARGTTSDAFDIWGQGTMVTVSSGGGGSGGGGSGGGGSDIQMTQSPSSLSASVGDRVTITCRASQSISSYLNWYQQKPGKAPKLLIDVASSLQSGVPSRFSGSGSGTDFTLTISSLQPEDFATYYCQQSYSTPLTFGGGTKVEIKRGQDASSAGSTRNKDPTRRPELEAGTNGRSSTTSPFVKPNPGSSTDGNSAGHSGNNILGSEVALFALMYVAAAAFVLLFFVGCGVLLSRKRRRMKLLSSIEQACDICRLKKLKCSKEKPKCAKCLKNNWECRYSPKTKRSPLTRAHLTEVESRLERLEQLFLLIFPREDLDMILKMDSLQDIKALLTGLFVQDNVNKDAVTDRLASVETDMPLTLRQHRISATSSSEESSNKGQRQLTVSAAAGGSGGSGGSDALDDFDLDMLGSDALDDFDLDMLGSDALDDFDLDMLGSDALDDFDLDMLGS

SEQ ID NO: 74 - DNA, 3274 bp, CLL1-synEphrinB2EC-NKG2D-CAR
aagcttgatatcgaattcggagcactgtcctccgaacgtcggagcactgtcctccgaacgtcggagcactgtcctccgaacgtcggagcactgtcctccgaacggagcatgtcctccgaacgtcggagcactgtcctccgaacgactagttaggcgtgtacggtgggaggcctatataagcagagctcgtttagtgaaccgtcagatcgcctggagacgccatccacgctgttttgacctccatagaagacaccgggaccgatccagcctctcgacattcgttggatcatgagagtgaagttcagcaggagcgcagacgcccccgcgtaccagcagggccagaaccagctctataacgagctcaatctaggacgaagagaggagtacgatgttttggacaagagacgtggccgggaccctgagatggggggaaagccgcagagaaggaagaaccctcaggaaggcctgtacaatgaactgcagaaagataagatggcggaggcctacagtgagattgggatgaaaggcgagcgccggaggggcaaggggcacgatggcctttaccagggtctcagtacagccaccaaggacacctacgacgcccttcacatgcaggccctgccccctcgcgggtggattcgtggtcggaggtctcgacacagctgggagatgagtgaatttcataattataacttggatctgaagaagagtgatttttcaacacgatggcaaaagcaaagatgtccagtagtcaaaagcaaatgtagagaaaatgcatctccattttttttctgctgcttcatcgctgtagccatgggaatccgtttcattattatggtagctatatggagtgctgtattcctaaactcattattcaaccaagaagttcaaattcccttgaccgaaagttactgtggcccatgtcctaaaaactggatatgttacaaaaataactgctaccaattttttgatgagagtaaaaactggtatgagagccaggcttcttgtatgtctcaaaatgccagccttctgaaagtatacagcaaagaggaccaggatttacttaaactggtgaagtcatatcattggatgggactagtacacattccaacaaatggatcttggcagtgggaagatggctccattctctcacccaacctactaacaataattgaaatgcagaagggagactgtgcactctatgcctcgagctttaaaggctatatagaaaactgttcaactccaaatacgtacatctgcatgcaaaggactgtgtaagctagcatcgatggctccggtgcccgtcagtgggcagagcgcacatcgcccacagtccccgagaagttggggggaggggtcggcaattgaaccggtgcctagagaaggtggcgcggggtaaactgggaaagtgatgtcgtgtactggctccgcctttttcccgagggtgggggagaaccgtatataagtgcagtagtcgccgtgaacgttctttttcgcaacgggtttgccgccagaacacaggtgtcgtgacgcggatccaggcctaagcttacgcgtcctagcgctaccggtcgccaccatggcgctccctgtcaccgcactgcttcttccgctggcactgctgctgcacgctgcacggcctgaggtgcagctggtgcagtctggggctgaggtgaagaagcctggggcctcagtgaaggtttcctgcaaggcatctggatacaccttcaacagctactatatgcactgggtgcgacaggcccctggacaagggcttgagtggatgggaatattcaaccctggtggtggtagcacaagctacgcacagaagttccagggcagagtcaccatgaccagggacacgtccacgagcacagtctacatggagctgagcagcctgagatctgaggacacggccgtgtattactgtgcgagaggaactacatccgatgcttttgatatctggggccaagggacaatggtcaccgtctcgagtggtggaggcggttcaggcggaggtggttctggcggtggcggatcggacatccagatgacccagtctccatcctccctgtctgcatctgtaggagacagagtcaccatcacttgccgggcaagtcagagcattagcagctatttaaattggtatcagcagaaaccagggaaagcccctaagctcctgatcgatgtcgcatccagtttgcaaagtggggtcccatcaaggttcagtggcagtggatctgggacagatttcactctcaccatcagcagtctgcaacctgaagattttgcaacttactactgtcaacagagttacagtacccctctcactttcggcggagggaccaaggtggagatcaaacgtggacaagatgcaagttctgctggatcaaccaggaataaagatccaacaagacgtccagaactagaagctggtacaaatggaagaagttcgacaacaagtccctttgtaaaaccaaatccaggttctagcacagacggcaacagcgccggacattcggggaacaacatcctcggttccgaagtggccttatttgcactcatgtacgtggcagcggccgccttcgtgctcctgttctttgtgggctgtggggtgctgctgtcccgcaagcgccggcggatgaagctgctgagcagcatcgagcaggcctgtgacatctgccggctgaagaaactgaagtgcagcaaagaaaagcccaagtgcgccaagtgcctgaagaacaactgggagtgccggtacagccccaagaccaagagaagccccctgaccagagcccacctgaccgaggtggaaagccggctggaaagactggaacagctgtttctgctgatcttcccacgcgaggacctggacatgatcctgaagatggacagcctgcaggacatcaaggccctgctgaccggcctgttcgtgcaggacaacgtgaacaaggacgccgtgaccgacagactggccagcgtggaaaccgacatgcccctgaccctgcggcagcacagaatcagcgccaccagcagcagcgaggaaagcagcaacaagggccagcggcagctgacagtgtctgctgctgcaggcggaagcggaggctctggcggatctgatgccctggacgacttcgacctggatatgctgggcagcgacgccctggatgattttgatctggacatgctgggatctgacgctctggacgatttcgatctcgacatgttgggatcagatgcactggatgactttgacctggacatgctcggatca

SEQ ID NO: 75 - protein, 45 aa, CD8 hinge region
TTTPAPRPPTPAPTIASQPLSLRPEACRPAAGGAVHTRGLDFACD

SEQ ID NO: 76 - protein, 24 aa, CD8 transmembrane region
IYIWAPLAGTCGVLLLSLVITLYC

SEQ ID NO: 77 - protein, 27 aa, CD28 transmembrane region
FWVLVVVGGVLACYSLLVTVAFIIFWV

SEQ ID NO: 78 - protein, 41 aa, CD28 intracellular region
RSKRSRLLHSDYMNMTPRRPGPTRKHYQPYAPPRDFAAYRS

SEQ ID NO: 79 - protein, 42 aa, 4-1BB
KRGRKKLLYIFKQPFMRPVQTTQEEDGCSCRFPEEEEGGCEL

SEQ ID NO: 80 - protein, 113 aa, CD3ζ
RVKFSRSADAPAYQQGQNQLYNELNLGRREEYDVLDKRRGRDPEMGGKPQRRKNPQEGLYNELQKDKMAEAYSEIGMKGERRRGKGHDGLYQGLSTATKDTYDALHMQALPPR

SEQ ID NO: 81 - protein, 21 aa, CD8αsignaling domain
MALPVTALLLPLALLLHAARP

SEQ ID NO: 82 - protein, 226 aa, 28Z
TTTPAPRPPTPAPTIASQPLSLRPEACRPAAGGAVHTRGLDFACDFWVLVVVGGVLACYSLLVTVAFIIFWVRSKRSRLLHSDYMNMTPRRPGPTRKHYQPYAPPRDFAAYRSRVKFSRSADAPAYQQGQNQLYNELNLGRREEYDVLDKRRGRDPEMGGKPQRRKNPQEGLYNELQKDKMAEAYSEIGMKGERRRGKGHDGLYQGLSTATKDTYDALHMQALPPR

SEQ ID NO: 83 - protein, 224 aa, BBZ
TTTPAPRPPTPAPTIASQPLSLRPEACRPAAGGAVHTRGLDFACDIYIWAPLAGTCGVLLLSLVITLYCKRGRKKLLYIFKQPFMRPVQTTQEEDGCSCRFPEEEEGGCELRVKFSRSADAPAYQQGQNQLYNELNLGRREEYDVLDKRRGRDPEMGGKPQRRKNPQEGLYNELQKDKMAEAYSEIGMKGERRRGKGHDGLYQGLSTATKDTYDALHMQALPPR

SEQ ID NO: 84 - protein, 268 aa, 28BBZ
TTTPAPRPPTPAPTIASQPLSLRPEACRPAAGGAVHTRGLDFACDFWVLVVVGGVLACYSLLVTVAFIIFWVRSKRSRLLHSDYMNMTPRRPGPTRKHYQPYAPPRDFAAYRSKRGRKKLLYIFKQPFMRPVQTTQEEDGCSCRFPEEEEGGCELRVKFSRSADAPAYQQGQNQLYNELNLGRREEYDVLDKRRGRDPEMGGKPQRRKNPQEGLYNELQKDKMAEAYSEIGMKGERRRGKGHDGLYQGLSTATKDTYDALHMQALPPR

SEQ ID NO: 85 - protein, 92 aa, Receptor regulatory domain of synEphrinB2EC-8
GQDASSAGSTRNKDPTRRPELEAGTNGRSSTTSPFVKPNPGSSTDGNSAGHSGNNILGSEVALFAFMYVAAAAFVLLFFVGCGVLLSRKRRR

SEQ ID NO: 86 - protein, 242 aa, anti CD123-scFv
EVQLLESGGGLVQPGGSLRLSCAASGFTFSSYAMSWVRQAPGKGLEWVSAISGSGGSTYYADSVKGRFTISRDNSKNTLYLQMNSLRAEDTAVYYCAKDDSFYGGFDYWGQGTLVTVSSGGGGSGGGGSGGGGSDIQMTQSPSTLSASVGDRVTITCRASQSISSWLAWYQQKPGKAPKLLIYDASSLESGVPSRFSGSGSGTEFTLTISSLQPDDFATYYCQQYSSYKYTFGQGTKVEIKR

SEQ ID NO: 87 - protein, 556 aa, Amino acid sequence of GPC3-EphrinB2EC(comprsing human synotch transmembrane region)
EQKLISEEDLEVQLVQSGAEVKKPGASVKVSCKASGYTFSDYEMHWVRQAPGQGLEWMGAIHPGSGDTAYNQRFKGRVTITADKSTSTAYMELSSLRSEDTAVYYCARFYSYAYWGQGTLVTVSAGGGGSGGGGSGGGGSDIVMTQTPLSLPVTPGEPASISCRSSQSLVHSNGNTYLQWYLQKPGQSPQLLIYKVSNRFSGVPDRFSGSGSGTDFTLKISRVEAEDVGVYYCSQSIYVPYTFGQGTKLEIKRGQDASSAGSTRNKDPTRRPELEAGTNGRSSTTSPFVKPNPGSSTDGNSAGHSGNNILGSEVALFAFMYVAAAAFVLLFFVGCGVLLSRKRRRMKLLSSIEQACDICRLKKLKCSKEKPKCAKCLKNNWECRYSPKTKRSPLTRAHLTEVESRLERLEQLFLLIFPREDLDMILKMDSLQDIKALLTGLFVQDNVNKDAVTDRLASVETDMPLTLRQHRISATSSSEESSNKGQRQLTVSAAAGGSGGSGGSDALDDFDLDMLGSDALDDFDLDMLGSDALDDFDLDMLGSDALDDFDLDMLGS

SEQ ID NO: 88 - DNA, 3277 bp, CD123-synEphrinB2EC-NKG2D-CAR
aagcttgatatcgaattcggagcactgtcctccgaacgtcggagcactgtcctccgaacgtcggagcactgtcctccgaacgtcggagcactgtcctccgaacggagcatgtcctccgaacgtcggagcactgtcctccgaacgactagttaggcgtgtacggtgggaggcctatataagcagagctcgtttagtgaaccgtcagatcgcctggagacgccatccacgctgttttgacctccatagaagacaccgggaccgatccagcctctcgacattcgttggatcatgagagtgaagttcagcaggagcgcagacgcccccgcgtaccagcagggccagaaccagctctataacgagctcaatctaggacgaagagaggagtacgatgttttggacaagagacgtggccgggaccctgagatggggggaaagccgcagagaaggaagaaccctcaggaaggcctgtacaatgaactgcagaaagataagatggcggaggcctacagtgagattgggatgaaaggcgagcgccggaggggcaaggggcacgatggcctttaccagggtctcagtacagccaccaaggacacctacgacgcccttcacatgcaggccctgccccctcgcgggtggattcgtggtcggaggtctcgacacagctgggagatgagtgaatttcataattataacttggatctgaagaagagtgatttttcaacacgatggcaaaagcaaagatgtccagtagtcaaaagcaaatgtagagaaaatgcatctccattttttttctgctgcttcatcgctgtagccatgggaatccgtttcattattatggtagctatatggagtgctgtattcctaaactcattattcaaccaagaagttcaaattcccttgaccgaaagttactgtggcccatgtcctaaaaactggatatgttacaaaaataactgctaccaattttttgatgagagtaaaaactggtatgagagccaggcttcttgtatgtctcaaaatgccagccttctgaaagtatacagcaaagaggaccaggatttacttaaactggtgaagtcatatcattggatgggactagtacacattccaacaaatggatcttggcagtgggaagatggctccattctctcacccaacctactaacaataattgaaatgcagaagggagactgtgcactctatgcctcgagctttaaaggctatatagaaaactgttcaactccaaatacgtacatctgcatgcaaaggactgtgtaagctagcatcgatggctccggtgcccgtcagtgggcagagcgcacatcgcccacagtccccgagaagttggggggaggggtcggcaattgaaccggtgcctagagaaggtggcgcggggtaaactgggaaagtgatgtcgtgtactggctccgcctttttcccgagggtgggggagaaccgtatataagtgcagtagtcgccgtgaacgttctttttcgcaacgggtttgccgccagaacacaggtgtcgtgacgcggatccaggcctaagcttacgcgtcctagcgctaccggtcgccaccatggccttaccagtgaccgccttgctcctgccgctggccttgctgctccacgccgccaggccggaggtgcaattgctggagtctgggggaggcttggtacagcctggggggtccctgagactctcctgtgcagcctccggattcacctttagcagttatgccatgagctgggtccgccaggctccagggaaggggctggagtgggtctcagctattagtggtagtggtggtagcacatactacgcagactccgtgaagggccggttcaccatctccagagacaattccaagaacacgctgtatctgcagatgaacagcctgagagccgaggacacggccgtatattactgtgcgaaagatgattctttctacggtggtttcgactactggggccaaggaaccctggtcaccgtctcgagtggtggaggcggttcaggcggaggtggttctggcggtggcggatcggacatccagatgacccagtctccttccaccctgtctgcatctgtaggagaccgtgtcaccatcacttgccgtgccagtcagagtattagtagctggttggcctggtatcagcagaaaccagggaaagcccctaagctcctgatctatgatgcctccagtttggaaagtggggtcccatcacgtttcagcggcagtggatccgggacagaattcactctcaccatcagcagcttgcagcctgatgattttgcaacttattactgccaacagtactcttcttacaaatacacgtttggccagggcaccaaagtcgagatcaagcgtggacaagatgcaagttctgctggatcaaccaggaataaagatccaacaagacgtccagaactagaagctggtacaaatggaagaagttcgacaacaagtccctttgtaaaaccaaatccaggttctagcacagacggcaacagcgccggacattcggggaacaacatcctcggttccgaagtggccttatttgcactcatgtacgtggcagcggccgccttcgtgctcctgttctttgtgggctgtggggtgctgctgtcccgcaagcgccggcggatgaagctgctgagcagcatcgagcaggcctgtgacatctgccggctgaagaaactgaagtgcagcaaagaaaagcccaagtgcgccaagtgcctgaagaacaactgggagtgccggtacagccccaagaccaagagaagccccctgaccagagcccacctgaccgaggtggaaagccggctggaaagactggaacagctgtttctgctgatcttcccacgcgaggacctggacatgatcctgaagatggacagcctgcaggacatcaaggccctgctgaccggcctgttcgtgcaggacaacgtgaacaaggacgccgtgaccgacagactggccagcgtggaaaccgacatgcccctgaccctgcggcagcacagaatcagcgccaccagcagcagcgaggaaagcagcaacaagggccagcggcagctgacagtgtctgctgctgcaggcggaagcggaggctctggcggatctgatgccctggacgacttcgacctggatatgctgggcagcgacgccctggatgattttgatctggacatgctgggatctgacgctctggacgatttcgatctcgacatgttgggatcagatgcactggatgactttgacctggacatgctcggatca

SEQ ID NO: 89 - protein, 238 aa, antiEGFRvIII-scFv2
DVQLQSGPSLVKPSQSLSLTCTVTGYSITSDFAWNWIRQFPGNKLEWMGYISYSGNTRYNPSLKSRISITRDTSKNQFFLQLNSVTIEDTATYYCVTAGRGFPYWGQGTLVTVSAGGGGSGGGGSGGGGSDILMTQSPSSMSVSLGDTVSITCHSSQDINSNIGWLQQRPGKSFKGLIYHGTNLDDEVPSRFSGSGSGADYSLTISSLESEDFADYYCVQYAQFPWTFGGGTKLEIKR

SEQ ID NO: 90 - protein, 241 aa, antiMesothelin-scFv2
MQVQLQQSGPELEKPGASVKLSCKASGYSFTGYTMNWVKQSHGKSLEWIGLITPYNGASSYNQKFRGKATLTVDKSSSTAYMDLLSLTSEDSAVYFCARGGYDGRGFDYWGQGTTVTVSSGGGGSGGGGSGGGGSDIELTQSPAIMSASPGEKVTMTCSASSSVSYMHWYQQKSGTSPKRWIYDTSKLASGVPGRFSGSGSGNSYSLTISSVEAEDDATYYCQQWGSHPLTFGAGTKLEIK

SEQ ID NO: 91 - protein, 252 aa, antiFAP-scFv2
QVQLVQSGAEVKKPGASVKVSCKTSRYTFTEYTIHWVRQAPGQRLEWIGGINPNNGIPNYNQKFKGRVTITVDTSASTAYMELSSLRSEDTAVYYCARRRIAYGYDEGHAMDYWGQGTLVTVSSGGGGSGGGGSGGGGSDIVMTQSPDSLAVSLGERATINCKSSQSLLYSRNQKNYLAWYQQKPGQPPKLLIFWASTRESGVPDRFSGSGFGTDFTLTISSLQAEDVAVYYCQQYFSYPLTFGQGTKVEIK

SEQ ID NO: 92 - protein, 227 aa, antiCLL1-scFv2
EVQLQQSGPELVKPGASVKMSCKASGYTFTSYFIHWVKQKPGQGLEWIKGKATLTADKSSSTAYMELSSLTSEDSAVYYCTRDDGYYGYAMDYWGQGTSVTVSSGGGGSGGGGSGGGGSDIQMTQSPSSLSASLGERVSLTCRATQELSGYLSWLQQKPDGTIKRLIYAASTLDSGVPKRFSGNRSGSDYSLTISSLESEDFADYYCLQYAIYPYTFGGGTKLEIKR

SEQ ID NO: 93 - protein, 245 aa, antiIL13Ra2-scFv1
EVQLLESGGGLVQPGGSLRLSCAASGFTFRKYAMGWVRQAPGKGLEWVSGISGSVGSTYYADSVKGRFTISRDNSKNTLYLQMNSLRAEDTAVYYCAKVRYGWGAGAFDYWGQGTLVTVSSGGGGSGGGGSGGGGSDIQMTQSPSTLSASVGDRVTITCRASQSISSWLAWYQQKPGKAPKLLIYDASSLESGVPSRFSGSGSGTEFTLTISSLQPDDFATYYCQQYDTYPPITFGQGTKVEIKR

SEQ ID NO: 94 - protein, 238 aa, antiIL13Ra2-scFv2
GPELKKPGETVKIYCKASGYSFRDYSVHWVKQAPGKGLKWMGWINTETGEPTYVDEFKGRFAFFLEASANTVYLQISNLKNEDTATYFCDYRFTYWGQGTLVTVSAAKGGGGSGGGGSGGGGSEIVMTQTPLILSVTIGQPASISCKSSQSVLYSNGKTYLNWLLQRPGQSPKRLIYLVSKLDSGVPDRFTGSGSGTDFTLKISRVEAEDLGVYYCVQGSHFPYTFGGGTKLEIKRAD

SEQ ID NO: 95 - protein, 243 aa, antiGPC3-scFv-2
DVVMTQSPLSLPVTPGEPASISCRSSQSLVHSNANTYLHWYLQKPGQSPQLLIYKVSNRFSGVPDRFSGSGSGTDFTLKISRVEAEDVGVYYCSQNTHVPPTFGQGTKLEIKRGGGGSGGGGSGGGGSQVQLVQSGAEVKKPGASVKVSCKASGYTFTDYEMHWVRQAPGQGLEWMGALDPKTGDTAYSQKFKGRVTLTADESTSTAYMELSSLRSEDTAVYYCTRFYSYTYWGQGTLVTVSS

SEQ ID NO: 96 - protein, 246 aa, anti Claudin18.2 scFv-2
QVQLQQPGAELVRPGASVKLSCKASGYTFTSYWINWVKQRPGQGLEWIGNIYPSDSYTNYNQKFKDKATLTVDKSSSTAYMQLSSPTSEDSAVYYCTRSWRGNSFDYWGQGTTLTVSSGGGGSGGGGSGGGGSDIVMTQSPSSLTVTAGEKVTMSCKSSQSLLNSGNQKNYLTWYQQKPGQPPKLLIYWASTRESGVPDRFTGSGSGTDFTLTISSVQAEDLAVYYCQNDYSYPFTFGSGTKLEIK

SEQ ID NO: 97 - protein, 247 aa, anti Claudin18.2 scFv-3
QIQLVQSGPELKKPGETVKISCKASGYTFTNYGMNWVKQAPGKGLKWMGWINTNTGEPTYAEEFKGRFAFSLETSASTAYLQINNLKNEDTATYFCARLGFGNAMDYWGQGTSVTVSSGGGGSGGGGSGGGGSDIVMTQSPSSLTVTAGEKVTMSCKSSQSLLNSGNQKNYLTWYQQKPGQPPKLLIYWASTRESGVPDRFTGSGSGTDFTLTISSVQAEDLAVYYCQNDYSYPLTFGAGTKLELKR

SEQ ID NO: 98 - protein, 247 aa, anti Claudin18.2 scFv-4
QVQLQQPGAELVRPGASVKLSCKASGYTFTSYWINWVKQRPGQGLEWIGNIYPSDSYTNYNQKFKDKATLTVDKSSSTAYMQLSSPTSEDSAVYYCTRSWRGNSFDYWGQGTTLTVSSGGGGSGGGGSGGGGSDIVMTQSPSSLTVTAGEKVTMSCKSSQSLLNSGNQKNYLTWYQQKPGQPPKLLIYWASTRESGVPDRFTGSGSGTDFTLTISSVQAEDLAVYYCQNDYSYPFTFGSGTKLEIKR

SEQ ID NO: 99 - protein, 241 aa, antiB7H3-scFv1
EVQLLESGGGLVQPGGSLRLSCAASGFTFSSYAMSWVRQAPGKGLEWVSAISGSGGSTYYADSVKGRFTISRDNSKNTLYLQMNSLRAEDTAVYYCAKYRAVTFDYWGQGTLVTVSSGGGGSGGGGSGGGGSDIQMTQSPSTLSASVGDRVTITCRASQSISSWLAWYQQKPGKAPKLLIYDASSLESGVPSRFSGSGSGTEFTLTISSLQPDDFATYYCQQFETQIRWTFGQGTKVEIKR

SEQ ID NO: 100 - protein, 240 aa, 376.96-scFv
DIVMTQSHKFMSTSIGARVSITCKASQDVRTAVAWYQQKPGQSPKLLIYSASYRYTGVPDRFTGSGSGTDFTFTISSVQAEDLAVYYCQQHYGTPPWTFGGGTKLEIKGGGGSGGGGSGGGGSEVQLVESGGGLVKPGGSLKLSCEASRFTFSSYAMSWVRQTPEKRLEWVAAISGGGRYTYYPDSMKGRFTISRDNAKNFLYLQMSSLRSEDTAMYYCARHYDGYLDYWGQGTTLTVSS

SEQ ID NO: 101 - protein, 244 aa, antiB7H3-scFv2
EVQLVESGGGLVQPGGSLRLSCAASGFTFSSFGMHWVRQAPGKGLEWVAYISSDSSAIYYADTVKGRFTISRDNAKNSLYLQMNSLRDEDTAVYYCGRGRENIYYGSRLDYWGQGTTVTVSSGGGGSGGGGSGGGGSDIQLTQSPSFLSASVGDRVTITCKASQNVDTNVAWYQQKPGKAPKALIYSASYRYSGVPSRFSGSGSGTDFTLTISSLQPEDFATYYCQQYNNYPFTFGQGTKLEIK

SEQ ID NO: 102 - protein, 28 aa, Notch1 transmembrane region(Notch2STS)
LMYVAAAAFVLLFFVGCGVLLSKRKRKH

SEQ ID NO: 103 - protein, 28 aa, Notch1 transmembrane region（Notch3STS）
LMYVAAAAFVLLFFVGCGVLLSRRKREH

SEQ ID NO: 104 - protein, 29 aa, Notch1 transmembrane region（Notch4STS）
LMYVAAAAFVLLFFVGCGVLLSRRRRREH

SEQ ID NO: 105 - protein, 550 aa, Amino acid sequence of Mesothelin-synEphrinB2EC
QMQLVQSGAEVKKPGASVKVSCKASGYTFTSYYMHWVRQAPGQGLEWMGIINPSGGSTSYAQKFQGRVTMTRDTSTSTVYMELSSLRSEDTAVYYCASSRSGTTVVNHDAFDIWGKGTTVTVSSGGGGSGGGGSGGGGSDIQLTQSPSSLSASVGDRVTITCRASQVISRALAWYQQTPGKPPKLLIYDASNLQSGVPSRFSGSGSGTDFTLTISRLQPEDFATYYCQQFNSYPLTFGGGTKLEIKRGQDASSAGSTRNKDPTRRPELEAGTNGRSSTTSPFVKPNPGSSTDGNSAGHSGNNILGSEVALFALMYVAAAAFVLLFFVGCGVLLSRKRRRMKLLSSIEQACDICRLKKLKCSKEKPKCAKCLKNNWECRYSPKTKRSPLTRAHLTEVESRLERLEQLFLLIFPREDLDMILKMDSLQDIKALLTGLFVQDNVNKDAVTDRLASVETDMPLTLRQHRISATSSSEESSNKGQRQLTVSAAAGGSGGSGGSDALDDFDLDMLGSDALDDFDLDMLGSDALDDFDLDMLGSDALDDFDLDMLGS

SEQ ID NO: 106 - protein, 547 aa, Amino acid sequence of FAP-synEphrinB2EC
QVQLVQSGAEVKKPGSSVKVSCKASGGTFSSYAISWVRQAPGQGLEWMGGIIPIFGTANYAQKFQGRVTITADKSTSTAYMELSSLRSEDTAVYYCARDAADRDYWGQGTTVTVSSGGGGSGGGGSGGGGSDIVMTQSPLSLPVTPGEPASISCRSSQSLLHPNGFNHLYWYLQKPGQSPQLLIYVGGNRASGVPDRFSGSGSGTDFTLKISRVEAEDVGVYYCQQRNNKNRTFGQGTKVEIKRGQDASSAGSTRNKDPTRRPELEAGTNGRSSTTSPFVKPNPGSSTDGNSAGHSGNNILGSEVALFALMYVAAAAFVLLFFVGCGVLLSRKRRRMKLLSSIEQACDICRLKKLKCSKEKPKCAKCLKNNWECRYSPKTKRSPLTRAHLTEVESRLERLEQLFLLIFPREDLDMILKMDSLQDIKALLTGLFVQDNVNKDAVTDRLASVETDMPLTLRQHRISATSSSEESSNKGQRQLTVSAAAGGSGGSGGSDALDDFDLDMLGSDALDDFDLDMLGSDALDDFDLDMLGSDALDDFDLDMLGS

SEQ ID NO: 107 - protein, 471 aa, Mesothelin-CAR
QMQLVQSGAEVKKPGASVKVSCKASGYTFTSYYMHWVRQAPGQGLEWMGIINPSGGSTSYAQKFQGRVTMTRDTSTSTVYMELSSLRSEDTAVYYCASSRSGTTVVNHDAFDIWGKGTTVTVSSGGGGSGGGGSGGGGSDIQLTQSPSSLSASVGDRVTITCRASQVISRALAWYQQTPGKPPKLLIYDASNLQSGVPSRFSGSGSGTDFTLTISRLQPEDFATYYCQQFNSYPLTFGGGTKLEIKRTTTPAPRPPTPAPTIASQPLSLRPEACRPAAGGAVHTRGLDFACDIYIWAPLAGTCGVLLLSLVITLYCKRGRKKLLYIFKQPFMRPVQTTQEEDGCSCRFPEEEEGGCELRVKFSRSADAPAYQQGQNQLYNELNLGRREEYDVLDKRRGRDPEMGGKPQRRKNPQEGLYNELQKDKMAEAYSEIGMKGERRRGKGHDGLYQGLSTATKDTYDALHMQALPPR

SEQ ID NO: 108 - protein, 550 aa, Claudin18.2-synEphrinB2EC
QVQLQESGPGLIKPSQTLSLTCTVSGGSISSGYNWHWIRQPPGKGLEWIGYIHYTGSTNYNPALRSRVTISVDTSKNQFSLKLSSVTAADTAIYYCARIYNGNSFPYWGQGTTVTVSSGGGGSGGGGSGGGGSDIVMTQSPDSLAVSLGERATINCKSSQSLFNSGNQKNYLTWYQQKPGQPPKLLIYWASTRESGVPDRFSGSGSGTDFTLTISSLQAEDVAVYYCQNAYSFPYTFGGGTKLEIKRGQDASSAGSTRNKDPTRRPELEAGTNGRSSTTSPFVKPNPGSSTDGNSAGHSGNNILGSEVALFALMYVAAAAFVLLFFVGCGVLLSRKRRRMKLLSSIEQACDICRLKKLKCSKEKPKCAKCLKNNWECRYSPKTKRSPLTRAHLTEVESRLERLEQLFLLIFPREDLDMILKMDSLQDIKALLTGLFVQDNVNKDAVTDRLASVETDMPLTLRQHRISATSSSEESSNKGQRQLTVSAAAGGSGGSGGSDALDDFDLDMLGSDALDDFDLDMLGSDALDDFDLDMLGSDALDDFDLDMLGS

SEQ ID NO: 109 - protein, 329 aa, NKG2D-CAR
MRVKFSRSADAPAYQQGQNQLYNELNLGRREEYDVLDKRRGRDPEMGGKPQRRKNPQEGLYNELQKDKMAEAYSEIGMKGERRRGKGHDGLYQGLSTATKDTYDALHMQALPPRGWIRGRRSRHSWEMSEFHNYNLDLKKSDFSTRWQKQRCPVVKSKCRENASPFFFCCFIAVAMGIRFIIMVAIWSAVFLNSLFNQEVQIPLTESYCGPCPKNWICYKNNCYQFFDESKNWYESQASCMSQNASLLKVYSKEDQDLLKLVKSYHWMGLVHIPTNGSWQWEDGSILSPNLLTIIEMQKGDCALYASSFKGYIENCSTPNTYICMQRTV

SEQ ID NO: 110 - protein, 545 aa, Amino acid sequence of CLL1-synEphrinB2EC-APLP2（TM）
EVQLVQSGAEVKKPGASVKVSCKASGYTFNSYYMHWVRQAPGQGLEWMGIFNPGGGSTSYAQKFQGRVTMTRDTSTSTVYMELSSLRSEDTAVYYCARGTTSDAFDIWGQGTMVTVSSGGGGSGGGGSGGGGSDIQMTQSPSSLSASVGDRVTITCRASQSISSYLNWYQQKPGKAPKLLIDVASSLQSGVPSRFSGSGSGTDFTLTISSLQPEDFATYYCQQSYSTPLTFGGGTKVEIKRGQDASSAGSTRNKDPTRRPELEAGTNGRSSTTSPFVKPNPGSSTDGNSAGHSGNNILGSEVALFASALIGLLVIAVAIATVIVISLVMLRKRQMKLLSSIEQACDICRLKKLKCSKEKPKCAKCLKNNWECRYSPKTKRSPLTRAHLTEVESRLERLEQLFLLIFPREDLDMILKMDSLQDIKALLTGLFVQDNVNKDAVTDRLASVETDMPLTLRQHRISATSSSEESSNKGQRQLTVSAAAGGSGGSGGSDALDDFDLDMLGSDALDDFDLDMLGSDALDDFDLDMLGSDALDDFDLDMLGS